European Patent Application EP 4 806 922 A2, published September 16, 2026. Title: Multi-Specific Antibodies Integrating Dual Immune Modulating Moieties and Uses Thereof in Immunotherapy. Applicant: Lyvgen Biopharma CO., LTD. Application US. The sequence listing filed with the application follows.

SEQUENCE LISTING (109 sequences)

SEQ ID NO: 1 - protein, 17 aa, synthetic construct
DKTHTCPPCPAPELLGP

SEQ ID NO: 2 - protein, 102 aa, synthetic construct
SVFLFPPKPKDTLMISRTPEVTCVVVDVSHEDPEVKFNWYVDGVEVHNAKTKPREEQYNSTYRVVSVLTVLHQDWLNGKEYKCKVSNKALGAPIEKTISKAK

SEQ ID NO: 3 - protein, 492 aa, synthetic construct
EVQLVESGGGLVQPGGSLRLSCAASGFTFSTYAMNWVRQAPGKGLEWVGRIRSKYNNYATYYADSVKGRFTISRDDSKNSLYLQMNSLKTEDTAVYYCVRHGNFGNSYVSWFAYWGQGTLVTVSSGGGGSDKTHTCPPCPAPELLGPSVFLFPPKPKDTLMISRTPEVTCVVVDVSHEDPEVKFNWYVDGVEVHNAKTKPREEQYNSTYRVVSVLTVLHQDWLNGKEYKCKVSNKALGAPIEKTISKAKGQPREPQVYTLPPSREEMTKNQVSLWCLVKGFYPSDIAVEWESNGQPENNYKTTPPVLDSDGSFFLYSKLTVDKSRWQQGNVFSCSVMHEALHNHYTQKSLSLSPGKGGGGSGGGGSGGGGSGGGGSQVQLVQSGAEVKKPGASVKVSCKASGYTFAGFEMHWVRQAPGQGLEWMGAIDPKTGGTDYNQKFKDRVTMTRDTSISTAYMELSRLRSDDTAVYYCARDLGYFDVWGQGTLVTVSS

SEQ ID NO: 4 - protein, 467 aa, synthetic construct
QAVVTQEPSLTVSPGGTVTLTCRSSTGAVTTSNYANWVQQKPGQAPRGLIGGTNKRAPWTPARFSGSLLGGKAALTITGAQAEDEADYYCALWYSNLWVFGGGTKLTVLGGGGSDKTHTCPPCPAPELLGPSVFLFPPKPKDTLMISRTPEVTCVVVDVSHEDPEVKFNWYVDGVEVHNAKTKPREEQYNSTYRVVSVLTVLHQDWLNGKEYKCKVSNKALGAPIEKTISKAKGQPREPQVYTLPPSREEMTKNQVSLSCAVKGFYPSDIAVEWESNGQPENNYKTTPPVLDSDGSFFLVSKLTVDKSRWQQGNVFSCSVMHEALHNRFTQKSLSLSPGKGGGGSGGGGSGGGGSGGGGSDIQMTQSPSSLSASVGDRVTITCRASQDIRSNLNWYQQKPGGAVKLLIYYTSRLHSGVPSRFSGSGSGTDYTLTISSLQPEDFATYFCQQSEKLPRTFGGGTKVEIR

SEQ ID NO: 5 - protein, 498 aa, synthetic construct
EVQLVESGGGLVQPGGSLRLSCAASGFTFSTYAMNWVRQAPGKGLEWVGRIRSKYNNYATYYADSVKGRFTISRDDSKNSLYLQMNSLKTEDTAVYYCVRHGNFGNSYVSWFAYWGQGTLVTVSSGGGGSDKTHTCPPCPAPELLGPSVFLFPPKPKDTLMISRTPEVTCVVVDVSHEDPEVKFNWYVDGVEVHNAKTKPREEQYNSTYRVVSVLTVLHQDWLNGKEYKCKVSNKALGAPIEKTISKAKGQPREPQVYTLPPSREEMTKNQVSLWCLVKGFYPSDIAVEWESNGQPENNYKTTPPVLDSDGSFFLYSKLTVDKSRWQQGNVFSCSVMHEALHNHYTQKSLSLSPGKGGGGSGGGGSGGGGSGGGGSQVQLVQSGAEVKKPGASVKVSCKASGYTFTDFWMSWVRQAPGQGLEWMGQIYPNTGTTHSNEKFKGRVTMTRDTSTSTVYMELSSLRSEDTAVYYCARSYHISTTPNWFAYWGQGTLVTVSS

SEQ ID NO: 6 - protein, 466 aa, synthetic construct
QAVVTQEPSLTVSPGGTVTLTCRSSTGAVTTSNYANWVQQKPGQAPRGLIGGTNKRAPWTPARFSGSLLGGKAALTITGAQAEDEADYYCALWYSNLWVFGGGTKLTVLGGGGSDKTHTCPPCPAPELLGPSVFLFPPKPKDTLMISRTPEVTCVVVDVSHEDPEVKFNWYVDGVEVHNAKTKPREEQYNSTYRVVSVLTVLHQDWLNGKEYKCKVSNKALGAPIEKTISKAKGQPREPQVYTLPPSREEMTKNQVSLSCAVKGFYPSDIAVEWESNGQPENNYKTTPPVLDSDGSFFLVSKLTVDKSRWQQGNVFSCSVMHEALHNRFTQKSLSLSPGKGGGGSGGGGSGGGGSGGGGSDIQMTQSPSSLSASVGDRVTITCKASQNVYKKLEWYQQKPGKVPKVLIYHTNILQTGVPSRFSGSGSGTDYTLTISSLQPEDVATYYCYQWNSGPTFGGGTKVEIK

SEQ ID NO: 7 - protein, 125 aa, synthetic construct
EVQLVESGGGLVQPGGSLRLSCAASGFTFSTYAMNWVRQAPGKGLEWVGRIRSKYNNYATYYADSVKGRFTISRDDSKNSLYLQMNSLKTEDTAVYYCVRHGNFGNSYVSWFAYWGQGTLVTVSS

SEQ ID NO: 8 - protein, 109 aa, synthetic construct
QAVVTQEPSLTVSPGGTVTLTCRSSTGAVTTSNYANWVQQKPGQAPRGLIGGTNKRAPWTPARFSGSLLGGKAALTITGAQAEDEADYYCALWYSNLWVFGGGTKLTVL

SEQ ID NO: 9 - protein, 116 aa, synthetic construct
QVQLVQSGAEVKKPGASVKVSCKASGYTFAGFEMHWVRQAPGQGLEWMGAIDPKTGGTDYNQKFKDRVTMTRDTSISTAYMELSRLRSDDTAVYYCARDLGYFDVWGQGTLVTVSS

SEQ ID NO: 10 - protein, 107 aa, synthetic construct
DIQMTQSPSSLSASVGDRVTITCRASQDIRSNLNWYQQKPGGAVKLLIYYTSRLHSGVPSRFSGSGSGTDYTLTISSLQPEDFATYFCQQSEKLPRTFGGGTKVEIR

SEQ ID NO: 11 - protein, 122 aa, synthetic construct
QVQLVQSGAEVKKPGASVKVSCKASGYTFTDFWMSWVRQAPGQGLEWMGQIYPNTGTTHSNEKFKGRVTMTRDTSTSTVYMELSSLRSEDTAVYYCARSYHISTTPNWFAYWGQGTLVTVSS

SEQ ID NO: 12 - protein, 106 aa, synthetic construct
DIQMTQSPSSLSASVGDRVTITCKASQNVYKKLEWYQQKPGKVPKVLIYHTNILQTGVPSRFSGSGSGTDYTLTISSLQPEDVATYYCYQWNSGPTFGGGTKVEIK

SEQ ID NO: 13 - protein, 119 aa, synthetic construct [sequence omitted]

SEQ ID NO: 14 - protein, 107 aa, synthetic construct [sequence omitted]

SEQ ID NO: 15 - protein, 120 aa, synthetic construct [sequence omitted]

SEQ ID NO: 16 - protein, 107 aa, synthetic construct [sequence omitted]

SEQ ID NO: 17 - protein, 121 aa, synthetic construct
EVQLVESGGGLVQPGGSLRLSCAASGFNIKDTYMHWVRQAPGKGLEWVARIDPANGNSKYADSVKGRFTISADTSKNTAYLQMNSLRAEDTAVYYCAPFGYYVSDYAMAYWGQGTLVTVSS

SEQ ID NO: 18 - protein, 111 aa, synthetic construct
DIQLTQSPSSLSASVGDRVTITCRAGESVDIFGVGFLHWYQQKPGKAPKLLIYRASNLESGVPSRFSGSGSRTDFTLTISSLQPEDFATYYCQQTNEDPYTFGQGTKVEIK

SEQ ID NO: 19 - protein, 121 aa, synthetic construct
QVQLVQSGAEVKKPGASVKVSCKASGYTFTNHIIHWVRQAPGQGLEWMGYINPYPGYHAYNEKFQGRATMTSDTSTSTVYMELSSLRSEDTAVYYCARDGYYRDTDVLDYWGQGTLVTVSS

SEQ ID NO: 20 - protein, 107 aa, synthetic construct
DIQMTQSPSSLSASVGDRVTITCQASQDISNYLNWYQQKPGKAPKLLIYYTSRLHTGVPSRFSGSGSGTDFTFTISSLEPEDIATYYCQQGNTLPWTFGQGTKVEIK

SEQ ID NO: 21 - protein, 121 aa, synthetic construct
QLQLQESGPGLVKPSETLSLTCTVSGGSISSGSYFWGWIRQPPGKGLEWIGSIYYSGITYYNPSLKSRVTISVDTSKNQFSLKLSSVTAADTAVYYCARHDGAVAGLFDYWGQGTLVTVSS

SEQ ID NO: 22 - protein, 108 aa, synthetic construct
SYVLTQPPSVSVAPGQTARITCGGNNIGSKSVHWYQQPPGQAPVVVVYDDSDRPSGIPERFSGSNSGNTATLTISRVEAGDEAVYYCQVWDSSSDHVVFGGGTKLTVL

SEQ ID NO: 23 - protein, 738 aa, synthetic construct
EVQLVESGGGLVQPGGSLRLSCAASGFTFTDYTMDWVRQAPGKGLEWVADVNPNSGGSIYNQRFKGRFTLSVDRSKNTLYLQMNSLRAEDTAVYYCARNLGPSFYFDYWGQGTLVTVSSASVAAPSVFIFPPSDEQLKSGTASVVCLLNNFYPREAKVQWKVDNALQSGNSQESVTEQDSKDSTYSLSSTLTLSKADYEKHKVYACEVTHQGLSSPVTKSFNRGECGGGGSGGGGSGGGGSGGGGSEVQLVESGGGLVQPGGSLRLSCAASGFTFSTYAMNWVRQAPGKGLEWVGRIRSKYNNYATYYADSVKGRFTISRDDSKNSLYLQMNSLKTEDTAVYYCVRHGNFGNSYVSWFAYWGQGTLVTVSSGGGGSDKTHTCPPCPAPELLGPSVFLFPPKPKDTLMISRTPEVTCVVVDVSHEDPEVKFNWYVDGVEVHNAKTKPREEQYNSTYRVVSVLTVLHQDWLNGKEYKCKVSNKALGAPIEKTISKAKGQPREPQVYTLPPSREEMTKNQVSLWCLVKGFYPSDIAVEWESNGQPENNYKTTPPVLDSDGSFFLYSKLTVDKSRWQQGNVFSCSVMHEALHNHYTQKSLSLSPGKGGGGSGGGGSGGGGSGGGGSQVQLVQSGAEVKKPGASVKVSCKASGYTFAGFEMHWVRQAPGQGLEWMGAIDPKTGGTDYNQKFKDRVTMTRDTSISTAYMELSRLRSDDTAVYYCARDLGYFDVWGQGTLVTVSS

SEQ ID NO: 24 - protein, 710 aa, synthetic construct
EVQLVESGGGLVQPGGSLRLSCAASGFNIKDTYIHWVRQAPGKGLEWVARIYPTNGYTRYADSVKGRFTISADTSKNTAYLQMNSLRAEDTAVYYCSRWGGDGFYAMDYWGQGTLVTVSSASTKGPSVFPLAPSSKSTSGGTAALGCLVKDYFPEPVTVSWNSGALTSGVHTFPAVLQSSGLYSLSSVVTVPSSSLGTQTYICNVNHKPSNTKVDKKVEPKSCGGGGSGGGGSGGGGSGGGGSQAVVTQEPSLTVSPGGTVTLTCRSSTGAVTTSNYANWVQQKPGQAPRGLIGGTNKRAPWTPARFSGSLLGGKAALTITGAQAEDEADYYCALWYSNLWVFGGGTKLTVLGGGGSDKTHTCPPCPAPELLGPSVFLFPPKPKDTLMISRTPEVTCVVVDVSHEDPEVKFNWYVDGVEVHNAKTKPREEQYNSTYRVVSVLTVLHQDWLNGKEYKCKVSNKALGAPIEKTISKAKGQPREPQVYTLPPSREEMTKNQVSLSCAVKGFYPSDIAVEWESNGQPENNYKTTPPVLDSDGSFFLVSKLTVDKSRWQQGNVFSCSVMHEALHNRFTQKSLSLSPGKGGGGSGGGGSGGGGSGGGGSDIQMTQSPSSLSASVGDRVTITCRASQDIRSNLNWYQQKPGGAVKLLIYYTSRLHSGVPSRFSGSGSGTDYTLTISSLQPEDFATYFCQQSEKLPRTFGGGTKVEIR

SEQ ID NO: 25 - protein, 212 aa, synthetic construct
DIQMTQSPSSLSASVGDRVTITCKASQDVSIGVAWYQQKPGKAPKLLIYSASYRYTGVPSRFSGSGSGTDFTLTISSLQPEDFATYYCQQYYIYPYTFGQGTKVEIKSSASTKGPSVFPLAPSSKSTSGGTAALGCLVKDYFPEPVTVSWNSGALTSGVHTFPAVLQSSGLYSLSSVVTVPSSSLGTQTYICNVNHKPSNTKVDKKVEPKSC

SEQ ID NO: 26 - protein, 214 aa, synthetic construct
DIQMTQSPSSLSASVGDRVTITCRASQDVNTAVAWYQQKPGKAPKLLIYSASFLYSGVPSRFSGSRSGTDFTLTISSLQPEDFATYYCQQHYTTPPTFGQGTKVEIKRTVAAPSVFIFPPSDEQLKSGTASVVCLLNNFYPREAKVQWKVDNALQSGNSQESVTEQDSKDSTYSLSSTLTLSKADYEKHKVYACEVTHQGLSSPVTKSFNRGEC

SEQ ID NO: 27 - protein, 744 aa, synthetic construct
EVQLVESGGGLVQPGGSLRLSCAASGFTFTDYTMDWVRQAPGKGLEWVADVNPNSGGSIYNQRFKGRFTLSVDRSKNTLYLQMNSLRAEDTAVYYCARNLGPSFYFDYWGQGTLVTVSSASVAAPSVFIFPPSDEQLKSGTASVVCLLNNFYPREAKVQWKVDNALQSGNSQESVTEQDSKDSTYSLSSTLTLSKADYEKHKVYACEVTHQGLSSPVTKSFNRGECGGGGSGGGGSGGGGSGGGGSEVQLVESGGGLVQPGGSLRLSCAASGFTFSTYAMNWVRQAPGKGLEWVGRIRSKYNNYATYYADSVKGRFTISRDDSKNSLYLQMNSLKTEDTAVYYCVRHGNFGNSYVSWFAYWGQGTLVTVSSGGGGSDKTHTCPPCPAPELLGPSVFLFPPKPKDTLMISRTPEVTCVVVDVSHEDPEVKFNWYVDGVEVHNAKTKPREEQYNSTYRVVSVLTVLHQDWLNGKEYKCKVSNKALGAPIEKTISKAKGQPREPQVYTLPPSREEMTKNQVSLWCLVKGFYPSDIAVEWESNGQPENNYKTTPPVLDSDGSFFLYSKLTVDKSRWQQGNVFSCSVMHEALHNHYTQKSLSLSPGKGGGGSGGGGSGGGGSGGGGSQVQLVQSGAEVKKPGASVKVSCKASGYTFTDFWMSWVRQAPGQGLEWMGQIYPNTGTTHSNEKFKGRVTMTRDTSTSTVYMELSSLRSEDTAVYYCARSYHISTTPNWFAYWGQGTLVTVSS

SEQ ID NO: 28 - protein, 709 aa, synthetic construct
EVQLVESGGGLVQPGGSLRLSCAASGFNIKDTYIHWVRQAPGKGLEWVARIYPTNGYTRYADSVKGRFTISADTSKNTAYLQMNSLRAEDTAVYYCSRWGGDGFYAMDYWGQGTLVTVSSASTKGPSVFPLAPSSKSTSGGTAALGCLVKDYFPEPVTVSWNSGALTSGVHTFPAVLQSSGLYSLSSVVTVPSSSLGTQTYICNVNHKPSNTKVDKKVEPKSCGGGGSGGGGSGGGGSGGGGSQAVVTQEPSLTVSPGGTVTLTCRSSTGAVTTSNYANWVQQKPGQAPRGLIGGTNKRAPWTPARFSGSLLGGKAALTITGAQAEDEADYYCALWYSNLWVFGGGTKLTVLGGGGSDKTHTCPPCPAPELLGPSVFLFPPKPKDTLMISRTPEVTCVVVDVSHEDPEVKFNWYVDGVEVHNAKTKPREEQYNSTYRVVSVLTVLHQDWLNGKEYKCKVSNKALGAPIEKTISKAKGQPREPQVYTLPPSREEMTKNQVSLSCAVKGFYPSDIAVEWESNGQPENNYKTTPPVLDSDGSFFLVSKLTVDKSRWQQGNVFSCSVMHEALHNRFTQKSLSLSPGKGGGGSGGGGSGGGGSGGGGSDIQMTQSPSSLSASVGDRVTITCKASQNVYKKLEWYQQKPGKVPKVLIYHTNILQTGVPSRFSGSGSGTDYTLTISSLQPEDVATYYCYQWNSGPTFGGGTKVEIK

SEQ ID NO: 29 - protein, 17 aa, synthetic construct
DKTHTCPPCPAPEAAGP

SEQ ID NO: 30 - protein, 119 aa, synthetic construct [sequence omitted]

SEQ ID NO: 31 - protein, 602 aa, synthetic construct
EVQLVESGGGLVQPGGSLRLSCAASGFTFTDYTMDWVRQAPGKGLEWVADVNPNSGGSIYNQRFKGRFTLSVDRSKNTLYLQMNSLRAEDTAVYYCARNLGPSFYFDYWGQGTLVTVSSASVAAPSVFIFPPSDEQLKSGTASVVCLLNNFYPREAKVQWKVDNALQSGNSQESVTEQDSKDSTYSLSSTLTLSKADYEKHKVYACEVTHQGLSSPVTKSFNRGECGGGGSGGGGSGGGGSGGGGSEVQLVESGGGLVQPGGSLRLSCAASGFTFSTYAMNWVRQAPGKGLEWVGRIRSKYNNYATYYADSVKGRFTISRDDSKNSLYLQMNSLKTEDTAVYYCVRHGNFGNSYVSWFAYWGQGTLVTVSSGGGGSDKTHTCPPCPAPELLGPSVFLFPPKPKDTLMISRTPEVTCVVVDVSHEDPEVKFNWYVDGVEVHNAKTKPREEQYNSTYRVVSVLTVLHQDWLNGKEYKCKVSNKALGAPIEKTISKAKGQPREPQVYTLPPSREEMTKNQVSLWCLVKGFYPSDIAVEWESNGQPENNYKTTPPVLDSDGSFFLYSKLTVDKSRWQQGNVFSCSVMHEALHNHYTQKSLSLSPGK

SEQ ID NO: 32 - protein, 583 aa, synthetic construct
EVQLVESGGGLVQPGGSLRLSCAASGFNIKDTYIHWVRQAPGKGLEWVARIYPTNGYTRYADSVKGRFTISADTSKNTAYLQMNSLRAEDTAVYYCSRWGGDGFYAMDYWGQGTLVTVSSASTKGPSVFPLAPSSKSTSGGTAALGCLVKDYFPEPVTVSWNSGALTSGVHTFPAVLQSSGLYSLSSVVTVPSSSLGTQTYICNVNHKPSNTKVDKKVEPKSCGGGGSGGGGSGGGGSGGGGSQAVVTQEPSLTVSPGGTVTLTCRSSTGAVTTSNYANWVQQKPGQAPRGLIGGTNKRAPWTPARFSGSLLGGKAALTITGAQAEDEADYYCALWYSNLWVFGGGTKLTVLGGGGSDKTHTCPPCPAPELLGPSVFLFPPKPKDTLMISRTPEVTCVVVDVSHEDPEVKFNWYVDGVEVHNAKTKPREEQYNSTYRVVSVLTVLHQDWLNGKEYKCKVSNKALGAPIEKTISKAKGQPREPQVYTLPPSREEMTKNQVSLSCAVKGFYPSDIAVEWESNGQPENNYKTTPPVLDSDGSFFLVSKLTVDKSRWQQGNVFSCSVMHEALHNRFTQKSLSLSPGK

SEQ ID NO: 33 - protein, 106 aa, synthetic construct [sequence omitted]

SEQ ID NO: 34 - protein, 121 aa, synthetic construct [sequence omitted]

SEQ ID NO: 35 - protein, 447 aa, synthetic construct
EVQLVESGGGLVQPGGSLRLSCAASGFNIKDTYIHWVRQAPGKGLEWVARIYPTNGYTRYADSVKGRFTISADTSKNTAYLQMNSLRAEDTAVYYCSRWGGDGFYAMDYWGQGTLVTVSSASTKGPSVFPLAPCSRSTSESTAALGCLVKDYFPEPVTVSWNSGALTSGVHTFPAVLQSSGLYSLSSVVTVPSSSLGTKTYTCNVDHKPSNTKVDKRVESKYGPPCPPCPAPEFLGGPSVFLFPPKPKDTLMISRTPEVTCVVVDVSQEDPEVQFNWYVDGVEVHNAKTKPREEQFNSTYRVVSVLTVLHQDWLNGKEYKCKVSNKGLPSSIEKTISKAKGQPREPQVYTLPPCQEEMTKNQVSLWCLVKGFYPSDIAVEWESNGQPENNYKTTPPVLDSDGSFFLYSKLTVDKSRWQEGNVFSCSVMHEALHNHYTQKSLSLSLGK

SEQ ID NO: 36 - protein, 571 aa, synthetic construct
QVQLVQSGAEVVKPGASVKVSCKASGYTFTSYYIHWVRQAPGQGLEWIGSIYPGNVNTNYAQKFQGRATLTVDTSISTAYMELSRLRSDDTAVYYCTRSHYGLDWNFDVWGKGTTVTVSSSQVQLVESGGGVVQPGRSLRLSCAASGFTFTKAWMHWVRQAPGKQLEWVAQIKDKSNSYATYYADSVKGRFTISRDDSKNTLYLQMNSLRAEDTAVYYCRGVYYALSPFDYWGQGTLVTVSSRTASTKGPSVFPLAPCSRSTSESTAALGCLVKDYFPEPVTVSWNSGALTSGVHTFPAVLQSSGLYSLSSVVTVPSSSLGTKTYTCNVDHKPSNTKVDKRVESKYGPPCPPCPAPEFLGGPSVFLFPPKPKDTLMISRTPEVTCVVVDVSQEDPEVQFNWYVDGVEVHNAKTKPREEQFNSTYRVVSVLTVLHQDWLNGKEYKCKVSNKGLPSSIEKTISKAKGQPREPQVCTLPPSQEEMTKNQVSLSCAVKGFYPSDIAVEWESNGQPENNYKTTPPVLDSDGSFFLVSKLTVDKSRWQEGNVFSCSVMHEALHNHYTQKSLSLSLGK

SEQ ID NO: 37 - protein, 109 aa, synthetic construct [sequence omitted]

SEQ ID NO: 38 - protein, 338 aa, synthetic construct
DIVMTQTPLSLSVTPGQPASISCKSSQSLVHNNANTYLSWYLQKPGQSPQSLIYKVSNRFSGVPDRFSGSGSGTDFTLKISRVEAEDVGVYYCGQGTQYPFTFGSGTKVEIKGQPKAAPDIQMTQSPSSLSASVGDRVTITCQASQNIYVWLNWYQQKPGKAPKLLIYKASNLHTGVPSRFSGSGSGTDFTLTISSLQPEDIATYYCQQGQTYPYTFGQGTKLEIKTKGPSRTVAAPSVFIFPPSDEQLKSGTASVVCLLNNFYPREAKVQWKVDNALQSGNSQESVTEQDSKDSTYSLSSTLTLSKADYEKHKVYACEVTHQGLSSPVTKSFNRGEC

SEQ ID NO: 39 - protein, 736 aa, synthetic construct
EVQLVESGGGLVQPGGSLRLSCAASGFNIKDTYMHWVRQAPGKGLEWVARIDPANGNSKYADSVKGRFTISADTSKNTAYLQMNSLRAEDTAVYYCAPFGYYVSDYAMAYWGQGTLVTVSSASTKGPSVFPLAPSSKSTSGGTAALGCLVKDYFPEPVTVSWNSGALTSGVHTFPAVLQSSGLYSLSSVVTVPSSSLGTQTYICNVNHKPSNTKVDKKVEPKSCGGGGSGGGGSGGGGSGGGGSEVQLVESGGGLVQPGGSLRLSCAASGFTFSTYAMNWVRQAPGKGLEWVGRIRSKYNNYATYYADSVKGRFTISRDDSKNSLYLQMNSLKTEDTAVYYCVRHGNFGNSYVSWFAYWGQGTLVTVSSGGGGSDKTHTCPPCPAPELLGPSVFLFPPKPKDTLMISRTPEVTCVVVDVSHEDPEVKFNWYVDGVEVHNAKTKPREEQYNSTYRVVSVLTVLHQDWLNGKEYKCKVSNKALGAPIEKTISKAKGQPREPQVYTLPPSREEMTKNQVSLWCLVKGFYPSDIAVEWESNGQPENNYKTTPPVLDSDGSFFLYSKLTVDKSRWQQGNVFSCSVMHEALHNHYTQKSLSLSPGKGGGGSGGGGSGGGGSGGGGSQVQLVQSGAEVKKPGASVKVSCKASGYTFAGFEMHWVRQAPGQGLEWMGAIDPKTGGTDYNQKFKDRVTMTRDTSISTAYMELSRLRSDDTAVYYCARDLGYFDVWGQGTLVTVSS

SEQ ID NO: 40 - protein, 711 aa, synthetic construct
EVQLVESGGGLVQPGGSLRLSCAASGFNIKDTYMHWVRQAPGKGLEWVARIDPANGNSKYADSVKGRFTISADTSKNTAYLQMNSLRAEDTAVYYCAPFGYYVSDYAMAYWGQGTLVTVSSASTKGPSVFPLAPSSKSTSGGTAALGCLVKDYFPEPVTVSWNSGALTSGVHTFPAVLQSSGLYSLSSVVTVPSSSLGTQTYICNVNHKPSNTKVDKKVEPKSCGGGGSGGGGSGGGGSGGGGSQAVVTQEPSLTVSPGGTVTLTCRSSTGAVTTSNYANWVQQKPGQAPRGLIGGTNKRAPWTPARFSGSLLGGKAALTITGAQAEDEADYYCALWYSNLWVFGGGTKLTVLGGGGSDKTHTCPPCPAPELLGPSVFLFPPKPKDTLMISRTPEVTCVVVDVSHEDPEVKFNWYVDGVEVHNAKTKPREEQYNSTYRVVSVLTVLHQDWLNGKEYKCKVSNKALGAPIEKTISKAKGQPREPQVYTLPPSREEMTKNQVSLSCAVKGFYPSDIAVEWESNGQPENNYKTTPPVLDSDGSFFLVSKLTVDKSRWQQGNVFSCSVMHEALHNRFTQKSLSLSPGKGGGGSGGGGSGGGGSGGGGSDIQMTQSPSSLSASVGDRVTITCRASQDIRSNLNWYQQKPGGAVKLLIYYTSRLHSGVPSRFSGSGSGTDYTLTISSLQPEDFATYFCQQSEKLPRTFGGGTKVEIR

SEQ ID NO: 41 - protein, 436 aa, synthetic construct
DIQLTQSPSSLSASVGDRVTITCRAGESVDIFGVGFLHWYQQKPGKAPKLLIYRASNLESGVPSRFSGSGSRTDFTLTISSLQPEDFATYYCQQTNEDPYTFGQGTKVEIKRTVAAPSVFIFPPSDEQLKSGTASVVCLLNNFYPREAKVQWKVDNALQSGNSQESVTEQDSKDSTYSLSSTLTLSKADYEKHKVYACEVTHQGLSSPVTKSFNRGECDIQLTQSPSSLSASVGDRVTITCRAGESVDIFGVGFLHWYQQKPGKAPKLLIYRASNLESGVPSRFSGSGSRTDFTLTISSLQPEDFATYYCQQTNEDPYTFGQGTKVEIKRTVAAPSVFIFPPSDEQLKSGTASVVCLLNNFYPREAKVQWKVDNALQSGNSQESVTEQDSKDSTYSLSSTLTLSKADYEKHKVYACEVTHQGLSSPVTKSFNRGEC

SEQ ID NO: 42 - protein, 694 aa, synthetic construct
QVQLVQSGAEVKKPGASVKVSCKASGYTFTEFGMNWVRQAPGQGLEWMGWINTKTGEATYVEEFKGRVTFTTDTSTSTAYMELRSLRSDDTAVYYCARWDFAYYVEAMDYWGQGTTVTVSSASTKGPSVFPLAPSSKSTSGGTAALGCLVKDYFPEPVTVSWNSGALTSGVHTFPAVLQSSGLYSLSSVVTVPSSSLGTQTYICNVNHKPSNTKVDKKVEPKSCDGGGGSGGGGSEVQLLESGGGLVQPGGSLRLSCAASGFTFSTYAMNWVRQAPGKGLEWVSRIRSKYNNYATYYADSVKGRFTISRDDSKNTLYLQMNSLRAEDTAVYYCVRHGNFGNSYVSWFAYWGQGTLVTVSSASVAAPSVFIFPPSDEQLKSGTASVVCLLNNFYPREAKVQWKVDNALQSGNSQESVTEQDSKDSTYSLSSTLTLSKADYEKHKVYACEVTHQGLSSPVTKSFNRGECDKTHTCPPCPAPEAAGGPSVFLFPPKPKDTLMISRTPEVTCVVVDVSHEDPEVKFNWYVDGVEVHNAKTKPREEQYNSTYRVVSVLTVLHQDWLNGKEYKCKVSNKALGAPIEKTISKAKGQPREPQVYTLPPCRDELTKNQVSLWCLVKGFYPSDIAVEWESNGQPENNYKTTPPVLDSDGSFFLYSKLTVDKSRWQQGNVFSCSVMHEALHNHYTQKSLSLSPGK

SEQ ID NO: 43 - protein, 451 aa, synthetic construct
QVQLVQSGAEVKKPGASVKVSCKASGYTFTEFGMNWVRQAPGQGLEWMGWINTKTGEATYVEEFKGRVTFTTDTSTSTAYMELRSLRSDDTAVYYCARWDFAYYVEAMDYWGQGTTVTVSSASTKGPSVFPLAPSSKSTSGGTAALGCLVKDYFPEPVTVSWNSGALTSGVHTFPAVLQSSGLYSLSSVVTVPSSSLGTQTYICNVNHKPSNTKVDKKVEPKSCDKTHTCPPCPAPEAAGGPSVFLFPPKPKDTLMISRTPEVTCVVVDVSHEDPEVKFNWYVDGVEVHNAKTKPREEQYNSTYRVVSVLTVLHQDWLNGKEYKCKVSNKALGAPIEKTISKAKGQPREPQVCTLPPSRDELTKNQVSLSCAVKGFYPSDIAVEWESNGQPENNYKTTPPVLDSDGSFFLVSKLTVDKSRWQQGNVFSCSVMHEALHNHYTQKSLSLSPGK

SEQ ID NO: 44 - protein, 214 aa, synthetic construct
QAVVTQEPSLTVSPGGTVTLTCGSSTGAVTTSNYANWVQEKPGQAFRGLIGGTNKRAPGTPARFSGSLLGGKAALTLSGAQPEDEAEYYCALWYSNLWVFGGGTKLTVLSSASTKGPSVFPLAPSSKSTSGGTAALGCLVKDYFPEPVTVSWNSGALTSGVHTFPAVLQSSGLYSLSSVVTVPSSSLGTQTYICNVNHKPSNTKVDKKVEPKSC

SEQ ID NO: 45 - protein, 215 aa, synthetic construct
DIQMTQSPSSLSASVGDRVTITCKASAAVGTYVAWYQQKPGKAPKLLIYSASYRKRGVPSRFSGSGSGTDFTLTISSLQPEDFATYYCHQYYTYPLFTFGQGTKLEIKRTVAAPSVFIFPPSDEQLKSGTASVVCLLNNFYPREAKVQWKVDNALQSGNSQESVTEQDSKDSTYSLSSTLTLSKADYEKHKVYACEVTHQGLSSPVTKSFNRGEC

SEQ ID NO: 46 - protein, 742 aa, synthetic construct
EVQLVESGGGLVQPGGSLRLSCAASGFNIKDTYMHWVRQAPGKGLEWVARIDPANGNSKYADSVKGRFTISADTSKNTAYLQMNSLRAEDTAVYYCAPFGYYVSDYAMAYWGQGTLVTVSSASTKGPSVFPLAPSSKSTSGGTAALGCLVKDYFPEPVTVSWNSGALTSGVHTFPAVLQSSGLYSLSSVVTVPSSSLGTQTYICNVNHKPSNTKVDKKVEPKSCGGGGSGGGGSGGGGSGGGGSEVQLVESGGGLVQPGGSLRLSCAASGFTFSTYAMNWVRQAPGKGLEWVGRIRSKYNNYATYYADSVKGRFTISRDDSKNSLYLQMNSLKTEDTAVYYCVRHGNFGNSYVSWFAYWGQGTLVTVSSGGGGSDKTHTCPPCPAPELLGPSVFLFPPKPKDTLMISRTPEVTCVVVDVSHEDPEVKFNWYVDGVEVHNAKTKPREEQYNSTYRVVSVLTVLHQDWLNGKEYKCKVSNKALGAPIEKTISKAKGQPREPQVYTLPPSREEMTKNQVSLWCLVKGFYPSDIAVEWESNGQPENNYKTTPPVLDSDGSFFLYSKLTVDKSRWQQGNVFSCSVMHEALHNHYTQKSLSLSPGKGGGGSGGGGSGGGGSGGGGSQVQLVQSGAEVKKPGASVKVSCKASGYTFTDFWMSWVRQAPGQGLEWMGQIYPNTGTTHSNEKFKGRVTMTRDTSTSTVYMELSSLRSEDTAVYYCARSYHISTTPNWFAYWGQGTLVTVSS

SEQ ID NO: 47 - protein, 710 aa, synthetic construct
EVQLVESGGGLVQPGGSLRLSCAASGFNIKDTYMHWVRQAPGKGLEWVARIDPANGNSKYADSVKGRFTISADTSKNTAYLQMNSLRAEDTAVYYCAPFGYYVSDYAMAYWGQGTLVTVSSASTKGPSVFPLAPSSKSTSGGTAALGCLVKDYFPEPVTVSWNSGALTSGVHTFPAVLQSSGLYSLSSVVTVPSSSLGTQTYICNVNHKPSNTKVDKKVEPKSCGGGGSGGGGSGGGGSGGGGSQAVVTQEPSLTVSPGGTVTLTCRSSTGAVTTSNYANWVQQKPGQAPRGLIGGTNKRAPWTPARFSGSLLGGKAALTITGAQAEDEADYYCALWYSNLWVFGGGTKLTVLGGGGSDKTHTCPPCPAPELLGPSVFLFPPKPKDTLMISRTPEVTCVVVDVSHEDPEVKFNWYVDGVEVHNAKTKPREEQYNSTYRVVSVLTVLHQDWLNGKEYKCKVSNKALGAPIEKTISKAKGQPREPQVYTLPPSREEMTKNQVSLSCAVKGFYPSDIAVEWESNGQPENNYKTTPPVLDSDGSFFLVSKLTVDKSRWQQGNVFSCSVMHEALHNRFTQKSLSLSPGKGGGGSGGGGSGGGGSGGGGSDIQMTQSPSSLSASVGDRVTITCKASQNVYKKLEWYQQKPGKVPKVLIYHTNILQTGVPSRFSGSGSGTDYTLTISSLQPEDVATYYCYQWNSGPTFGGGTKVEIK

SEQ ID NO: 48 - protein, 118 aa, synthetic construct [sequence omitted]

SEQ ID NO: 49 - protein, 600 aa, synthetic construct
EVQLVESGGGLVQPGGSLRLSCAASGFNIKDTYMHWVRQAPGKGLEWVARIDPANGNSKYADSVKGRFTISADTSKNTAYLQMNSLRAEDTAVYYCAPFGYYVSDYAMAYWGQGTLVTVSSASTKGPSVFPLAPSSKSTSGGTAALGCLVKDYFPEPVTVSWNSGALTSGVHTFPAVLQSSGLYSLSSVVTVPSSSLGTQTYICNVNHKPSNTKVDKKVEPKSCGGGGSGGGGSGGGGSGGGGSEVQLVESGGGLVQPGGSLRLSCAASGFTFSTYAMNWVRQAPGKGLEWVGRIRSKYNNYATYYADSVKGRFTISRDDSKNSLYLQMNSLKTEDTAVYYCVRHGNFGNSYVSWFAYWGQGTLVTVSSGGGGSDKTHTCPPCPAPELLGPSVFLFPPKPKDTLMISRTPEVTCVVVDVSHEDPEVKFNWYVDGVEVHNAKTKPREEQYNSTYRVVSVLTVLHQDWLNGKEYKCKVSNKALGAPIEKTISKAKGQPREPQVYTLPPSREEMTKNQVSLWCLVKGFYPSDIAVEWESNGQPENNYKTTPPVLDSDGSFFLYSKLTVDKSRWQQGNVFSCSVMHEALHNHYTQKSLSLSPGK

SEQ ID NO: 50 - protein, 584 aa, synthetic construct
EVQLVESGGGLVQPGGSLRLSCAASGFNIKDTYMHWVRQAPGKGLEWVARIDPANGNSKYADSVKGRFTISADTSKNTAYLQMNSLRAEDTAVYYCAPFGYYVSDYAMAYWGQGTLVTVSSASTKGPSVFPLAPSSKSTSGGTAALGCLVKDYFPEPVTVSWNSGALTSGVHTFPAVLQSSGLYSLSSVVTVPSSSLGTQTYICNVNHKPSNTKVDKKVEPKSCGGGGSGGGGSGGGGSGGGGSQAVVTQEPSLTVSPGGTVTLTCRSSTGAVTTSNYANWVQQKPGQAPRGLIGGTNKRAPWTPARFSGSLLGGKAALTITGAQAEDEADYYCALWYSNLWVFGGGTKLTVLGGGGSDKTHTCPPCPAPELLGPSVFLFPPKPKDTLMISRTPEVTCVVVDVSHEDPEVKFNWYVDGVEVHNAKTKPREEQYNSTYRVVSVLTVLHQDWLNGKEYKCKVSNKALGAPIEKTISKAKGQPREPQVYTLPPSREEMTKNQVSLSCAVKGFYPSDIAVEWESNGQPENNYKTTPPVLDSDGSFFLVSKLTVDKSRWQQGNVFSCSVMHEALHNRFTQKSLSLSPGK

SEQ ID NO: 51 - protein, 107 aa, synthetic construct [sequence omitted]

SEQ ID NO: 52 - protein, 586 aa, synthetic construct
EVQLVESGGGLVQPGGSLRLSCAASGFNIKDTYMHWVRQAPGKGLEWVARIDPANGNSKYADSVKGRFTISADTSKNTAYLQMNSLRAEDTAVYYCAPFGYYVSDYAMAYWGQGTLVTVSSASTKGPSVFPLAPSSKSTSGGTAALGCLVKDYFPEPVTVSWNSGALTSGVHTFPAVLQSSGLYSLSSVVTVPSSSLGTQTYICNVNHKPSNTKVDKKVEPKSCDKTHTCPPCPAPELLGPSVFLFPPKPKDTLMISRTPEVTCVVVDVSHEDPEVKFNWYVDGVEVHNAKTKPREEQYNSTYRVVSVLTVLHQDWLNGKEYKCKVSNKALGAPIEKTISKAKGQPREPQVYTLPPSREEMTKNQVSLWCLVKGFYPSDIAVEWESNGQPENNYKTTPPVLDSDGSFFLYSKLTVDKSRWQQGNVFSCSVMHEALHNHYTQKSLSLSPGKGGGGSGGGGSGGGGSGGGGSQVQLVQSGAEVKKPGASVKVSCKASGYTFAGFEMHWVRQAPGQGLEWMGAIDPKTGGTDYNQKFKDRVTMTRDTSISTAYMELSRLRSDDTAVYYCARDLGYFDVWGQGTLVTVSS

SEQ ID NO: 53 - protein, 577 aa, synthetic construct
EVQLVESGGGLVQPGGSLRLSCAASGFNIKDTYMHWVRQAPGKGLEWVARIDPANGNSKYADSVKGRFTISADTSKNTAYLQMNSLRAEDTAVYYCAPFGYYVSDYAMAYWGQGTLVTVSSASTKGPSVFPLAPSSKSTSGGTAALGCLVKDYFPEPVTVSWNSGALTSGVHTFPAVLQSSGLYSLSSVVTVPSSSLGTQTYICNVNHKPSNTKVDKKVEPKSCDKTHTCPPCPAPELLGPSVFLFPPKPKDTLMISRTPEVTCVVVDVSHEDPEVKFNWYVDGVEVHNAKTKPREEQYNSTYRVVSVLTVLHQDWLNGKEYKCKVSNKALGAPIEKTISKAKGQPREPQVYTLPPSREEMTKNQVSLSCAVKGFYPSDIAVEWESNGQPENNYKTTPPVLDSDGSFFLVSKLTVDKSRWQQGNVFSCSVMHEALHNRFTQKSLSLSPGKGGGGSGGGGSGGGGSGGGGSDIQMTQSPSSLSASVGDRVTITCRASQDIRSNLNWYQQKPGGAVKLLIYYTSRLHSGVPSRFSGSGSGTDYTLTISSLQPEDFATYFCQQSEKLPRTFGGGTKVEIR

SEQ ID NO: 54 - protein, 735 aa, synthetic construct
EVQLVESGGGLVQPGGSLRLSCAASGFNIKDTYIHWVRQAPGKDLEWVARIYPTNGYTRYADSVKGRFTISADTSKNTAYLQMNSLRAEDTAVYYCSRWGGDGFYAMDYWGRGTLVTVSSASTKGPSVFPLAPSSKSTSGGTAALGCLVRDYFPEPVTVSWNSGALTSGVRTCPAVLQSSGLYSLSSVVTVPSSSLGTQTYICNVNHKPSNTKVDKKVEPKSCGGGGSGGGGSGGGGSGGGGSEVQLVESGGGLVQPGGSLRLSCAASGFTFSTYAMNWVRQAPGKGLEWVGRIRSKYNNYATYYADSVKGRFTISRDDSKNSLYLQMNSLKTEDTAVYYCVRHGNFGNSYVSWFAYWGQGTLVTVSSGGGGSDKTHTCPPCPAPELLGPSVFLFPPKPKDTLMISRTPEVTCVVVDVSHEDPEVKFNWYVDGVEVHNAKTKPREEQYNSTYRVVSVLTVLHQDWLNGKEYKCKVSNKALGAPIEKTISKAKGQPREPQVYTLPPSREEMTKNQVSLWCLVKGFYPSDIAVEWESNGQPENNYKTTPPVLDSDGSFFLYSKLTVDKSRWQQGNVFSCSVMHEALHNHYTQKSLSLSPGKGGGGSGGGGSGGGGSGGGGSQVQLVQSGAEVKKPGASVKVSCKASGYTFAGFEMHWVRQAPGQGLEWMGAIDPKTGGTDYNQKFKDRVTMTRDTSISTAYMELSRLRSDDTAVYYCARDLGYFDVWGQGTLVTVSS

SEQ ID NO: 55 - protein, 736 aa, synthetic construct
QVQLVQSGAEVKKPGASVKVSCKASGYTFTNHIIHWVRQAPGQGLEWMGYINPYPGYHAYNEKFQGRATMTSDTSTSTVYMELSSLRSEDTAVYYCARDGYYRDTDVLDYWGQGTLVTVSSASTKGPSVFPLAPSSKSTSGGTAALGCLVKDYFPEPVTVSWNSGALTSGVHTFPAVLQSSGLYSLSSVVTVPSSSLGTQTYICNVNHKPSNTKVDKKVEPKSCGGGGSGGGGSGGGGSGGGGSEVQLVESGGGLVQPGGSLRLSCAASGFTFSTYAMNWVRQAPGKGLEWVGRIRSKYNNYATYYADSVKGRFTISRDDSKNSLYLQMNSLKTEDTAVYYCVRHGNFGNSYVSWFAYWGQGTLVTVSSGGGGSDKTHTCPPCPAPELLGPSVFLFPPKPKDTLMISRTPEVTCVVVDVSHEDPEVKFNWYVDGVEVHNAKTKPREEQYNSTYRVVSVLTVLHQDWLNGKEYKCKVSNKALGAPIEKTISKAKGQPREPQVYTLPPSREEMTKNQVSLWCLVKGFYPSDIAVEWESNGQPENNYKTTPPVLDSDGSFFLYSKLTVDKSRWQQGNVFSCSVMHEALHNHYTQKSLSLSPGKGGGGSGGGGSGGGGSGGGGSQVQLVQSGAEVKKPGASVKVSCKASGYTFAGFEMHWVRQAPGQGLEWMGAIDPKTGGTDYNQKFKDRVTMTRDTSISTAYMELSRLRSDDTAVYYCARDLGYFDVWGQGTLVTVSS

SEQ ID NO: 56 - protein, 711 aa, synthetic construct
QVQLVQSGAEVKKPGASVKVSCKASGYTFTNHIIHWVRQAPGQGLEWMGYINPYPGYHAYNEKFQGRATMTSDTSTSTVYMELSSLRSEDTAVYYCARDGYYRDTDVLDYWGQGTLVTVSSASTKGPSVFPLAPSSKSTSGGTAALGCLVKDYFPEPVTVSWNSGALTSGVHTFPAVLQSSGLYSLSSVVTVPSSSLGTQTYICNVNHKPSNTKVDKKVEPKSCGGGGSGGGGSGGGGSGGGGSQAVVTQEPSLTVSPGGTVTLTCRSSTGAVTTSNYANWVQQKPGQAPRGLIGGTNKRAPWTPARFSGSLLGGKAALTITGAQAEDEADYYCALWYSNLWVFGGGTKLTVLGGGGSDKTHTCPPCPAPELLGPSVFLFPPKPKDTLMISRTPEVTCVVVDVSHEDPEVKFNWYVDGVEVHNAKTKPREEQYNSTYRVVSVLTVLHQDWLNGKEYKCKVSNKALGAPIEKTISKAKGQPREPQVYTLPPSREEMTKNQVSLSCAVKGFYPSDIAVEWESNGQPENNYKTTPPVLDSDGSFFLVSKLTVDKSRWQQGNVFSCSVMHEALHNRFTQKSLSLSPGKGGGGSGGGGSGGGGSGGGGSDIQMTQSPSSLSASVGDRVTITCRASQDIRSNLNWYQQKPGGAVKLLIYYTSRLHSGVPSRFSGSGSGTDYTLTISSLQPEDFATYFCQQSEKLPRTFGGGTKVEIR

SEQ ID NO: 57 - protein, 214 aa, synthetic construct
DIQMTQSPSSLSASVGDRVTITCQASQDISNYLNWYQQKPGKAPKLLIYYTSRLHTGVPSRFSGSGSGTDFTFTISSLEPEDIATYYCQQGNTLPWTFGQGTKVEIKRTVAAPSVFIFPPSDEQLKSGTASVVCLLNNFYPREAKVQWKVDNALQSGNSQESVTEQDSKDSTYSLSSTLTLSKADYEKHKVYACEVTHQGLSSPVTKSFNRGEC

SEQ ID NO: 58 - protein, 736 aa, synthetic construct
QLQLQESGPGLVKPSETLSLTCTVSGGSISSGSYFWGWIRQPPGKGLEWIGSIYYSGITYYNPSLKSRVTISVDTSKNQFSLKLSSVTAADTAVYYCARHDGAVAGLFDYWGQGTLVTVSSASTKGPSVFPLAPSSKSTSGGTAALGCLVKDYFPEPVTVSWNSGALTSGVHTFPAVLQSSGLYSLSSVVTVPSSSLGTQTYICNVNHKPSNTKVDKKVEPKSCGGGGSGGGGSGGGGSGGGGSEVQLVESGGGLVQPGGSLRLSCAASGFTFSTYAMNWVRQAPGKGLEWVGRIRSKYNNYATYYADSVKGRFTISRDDSKNSLYLQMNSLKTEDTAVYYCVRHGNFGNSYVSWFAYWGQGTLVTVSSGGGGSDKTHTCPPCPAPELLGPSVFLFPPKPKDTLMISRTPEVTCVVVDVSHEDPEVKFNWYVDGVEVHNAKTKPREEQYNSTYRVVSVLTVLHQDWLNGKEYKCKVSNKALGAPIEKTISKAKGQPREPQVYTLPPSREEMTKNQVSLWCLVKGFYPSDIAVEWESNGQPENNYKTTPPVLDSDGSFFLYSKLTVDKSRWQQGNVFSCSVMHEALHNHYTQKSLSLSPGKGGGGSGGGGSGGGGSGGGGSQVQLVQSGAEVKKPGASVKVSCKASGYTFAGFEMHWVRQAPGQGLEWMGAIDPKTGGTDYNQKFKDRVTMTRDTSISTAYMELSRLRSDDTAVYYCARDLGYFDVWGQGTLVTVSS

SEQ ID NO: 59 - protein, 711 aa, synthetic construct
QLQLQESGPGLVKPSETLSLTCTVSGGSISSGSYFWGWIRQPPGKGLEWIGSIYYSGITYYNPSLKSRVTISVDTSKNQFSLKLSSVTAADTAVYYCARHDGAVAGLFDYWGQGTLVTVSSASTKGPSVFPLAPSSKSTSGGTAALGCLVKDYFPEPVTVSWNSGALTSGVHTFPAVLQSSGLYSLSSVVTVPSSSLGTQTYICNVNHKPSNTKVDKKVEPKSCGGGGSGGGGSGGGGSGGGGSQAVVTQEPSLTVSPGGTVTLTCRSSTGAVTTSNYANWVQQKPGQAPRGLIGGTNKRAPWTPARFSGSLLGGKAALTITGAQAEDEADYYCALWYSNLWVFGGGTKLTVLGGGGSDKTHTCPPCPAPELLGPSVFLFPPKPKDTLMISRTPEVTCVVVDVSHEDPEVKFNWYVDGVEVHNAKTKPREEQYNSTYRVVSVLTVLHQDWLNGKEYKCKVSNKALGAPIEKTISKAKGQPREPQVYTLPPSREEMTKNQVSLSCAVKGFYPSDIAVEWESNGQPENNYKTTPPVLDSDGSFFLVSKLTVDKSRWQQGNVFSCSVMHEALHNRFTQKSLSLSPGKGGGGSGGGGSGGGGSGGGGSDIQMTQSPSSLSASVGDRVTITCRASQDIRSNLNWYQQKPGGAVKLLIYYTSRLHSGVPSRFSGSGSGTDYTLTISSLQPEDFATYFCQQSEKLPRTFGGGTKVEIR

SEQ ID NO: 60 - protein, 214 aa, synthetic construct
SYVLTQPPSVSVAPGQTARITCGGNNIGSKSVHWYQQPPGQAPVVVVYDDSDRPSGIPERFSGSNSGNTATLTISRVEAGDEAVYYCQVWDSSSDHVVFGGGTKLTVLGQPKAAPSVTLFPPSSEELQANKATLVCLISDFYPGAVTVAWKGDSSPVKAGVETTTPSKQSNNKYAASSYLSLTPEQWKSHRSYSCQVTHEGSTVEKTVAPTECS

SEQ ID NO: 61 - protein, 600 aa, synthetic construct
QLQLQESGPGLVKPSETLSLTCTVSGGSISSGSYFWGWIRQPPGKGLEWIGSIYYSGITYYNPSLKSRVTISVDTSKNQFSLKLSSVTAADTAVYYCARHDGAVAGLFDYWGQGTLVTVSSASTKGPSVFPLAPSSKSTSGGTAALGCLVKDYFPEPVTVSWNSGALTSGVHTFPAVLQSSGLYSLSSVVTVPSSSLGTQTYICNVNHKPSNTKVDKKVEPKSCGGGGSGGGGSGGGGSGGGGSEVQLVESGGGLVQPGGSLRLSCAASGFTFSTYAMNWVRQAPGKGLEWVGRIRSKYNNYATYYADSVKGRFTISRDDSKNSLYLQMNSLKTEDTAVYYCVRHGNFGNSYVSWFAYWGQGTLVTVSSGGGGSDKTHTCPPCPAPELLGPSVFLFPPKPKDTLMISRTPEVTCVVVDVSHEDPEVKFNWYVDGVEVHNAKTKPREEQYNSTYRVVSVLTVLHQDWLNGKEYKCKVSNKALGAPIEKTISKAKGQPREPQVYTLPPSREEMTKNQVSLWCLVKGFYPSDIAVEWESNGQPENNYKTTPPVLDSDGSFFLYSKLTVDKSRWQQGNVFSCSVMHEALHNHYTQKSLSLSPGK

SEQ ID NO: 62 - protein, 584 aa, synthetic construct
QLQLQESGPGLVKPSETLSLTCTVSGGSISSGSYFWGWIRQPPGKGLEWIGSIYYSGITYYNPSLKSRVTISVDTSKNQFSLKLSSVTAADTAVYYCARHDGAVAGLFDYWGQGTLVTVSSASTKGPSVFPLAPSSKSTSGGTAALGCLVKDYFPEPVTVSWNSGALTSGVHTFPAVLQSSGLYSLSSVVTVPSSSLGTQTYICNVNHKPSNTKVDKKVEPKSCGGGGSGGGGSGGGGSGGGGSQAVVTQEPSLTVSPGGTVTLTCRSSTGAVTTSNYANWVQQKPGQAPRGLIGGTNKRAPWTPARFSGSLLGGKAALTITGAQAEDEADYYCALWYSNLWVFGGGTKLTVLGGGGSDKTHTCPPCPAPELLGPSVFLFPPKPKDTLMISRTPEVTCVVVDVSHEDPEVKFNWYVDGVEVHNAKTKPREEQYNSTYRVVSVLTVLHQDWLNGKEYKCKVSNKALGAPIEKTISKAKGQPREPQVYTLPPSREEMTKNQVSLSCAVKGFYPSDIAVEWESNGQPENNYKTTPPVLDSDGSFFLVSKLTVDKSRWQQGNVFSCSVMHEALHNRFTQKSLSLSPGK

SEQ ID NO: 63 - protein, 709 aa, synthetic construct
EVQLVESGGGLVQPGGSLRLSCAASGFTFTDYTMDWVRQAPGKRLEWVADVNPNSGGSIYNQRFKGRFTLSVDRSKNTLYLQMNSLRAEDTAVYYCARNLGPSFYFDYWGDGTLVTVSSASTKGPSVFPLAPSSKSTSGGTAALGCLVDDYFPEPVTVSWNSGALTSGVDTFPAVLQSSGLYSLCSVVTVPSSSLGTQTYICNVNHKPSNTKVDKKVEPKSCGGGGSGGGGSGGGGSGGGGSQAVVTQEPSLTVSPGGTVTLTCRSSTGAVTTSNYANWVQQKPGQAPRGLIGGTNKRAPWTPARFSGSLLGGKAALTITGAQAEDEADYYCALWYSNLWVFGGGTKLTVLGGGGSDKTHTCPPCPAPELLGPSVFLFPPKPKDTLMISRTPEVTCVVVDVSHEDPEVKFNWYVDGVEVHNAKTKPREEQYNSTYRVVSVLTVLHQDWLNGKEYKCKVSNKALGAPIEKTISKAKGQPREPQVYTLPPSREEMTKNQVSLSCAVKGFYPSDIAVEWESNGQPENNYKTTPPVLDSDGSFFLVSKLTVDKSRWQQGNVFSCSVMHEALHNRFTQKSLSLSPGKGGGGSGGGGSGGGGSGGGGSDIQMTQSPSSLSASVGDRVTITCRASQDIRSNLNWYQQKPGGAVKLLIYYTSRLHSGVPSRFSGSGSGTDYTLTISSLQPEDFATYFCQQSEKLPRTFGGGTKVEIR

SEQ ID NO: 64 - protein, 586 aa, synthetic construct
QLQLQESGPGLVKPSETLSLTCTVSGGSISSGSYFWGWIRQPPGKGLEWIGSIYYSGITYYNPSLKSRVTISVDTSKNQFSLKLSSVTAADTAVYYCARHDGAVAGLFDYWGQGTLVTVSSASTKGPSVFPLAPSSKSTSGGTAALGCLVKDYFPEPVTVSWNSGALTSGVHTFPAVLQSSGLYSLSSVVTVPSSSLGTQTYICNVNHKPSNTKVDKKVEPKSCDKTHTCPPCPAPELLGPSVFLFPPKPKDTLMISRTPEVTCVVVDVSHEDPEVKFNWYVDGVEVHNAKTKPREEQYNSTYRVVSVLTVLHQDWLNGKEYKCKVSNKALGAPIEKTISKAKGQPREPQVYTLPPSREEMTKNQVSLWCLVKGFYPSDIAVEWESNGQPENNYKTTPPVLDSDGSFFLYSKLTVDKSRWQQGNVFSCSVMHEALHNHYTQKSLSLSPGKGGGGSGGGGSGGGGSGGGGSQVQLVQSGAEVKKPGASVKVSCKASGYTFAGFEMHWVRQAPGQGLEWMGAIDPKTGGTDYNQKFKDRVTMTRDTSISTAYMELSRLRSDDTAVYYCARDLGYFDVWGQGTLVTVSS

SEQ ID NO: 65 - protein, 577 aa, synthetic construct
QLQLQESGPGLVKPSETLSLTCTVSGGSISSGSYFWGWIRQPPGKGLEWIGSIYYSGITYYNPSLKSRVTISVDTSKNQFSLKLSSVTAADTAVYYCARHDGAVAGLFDYWGQGTLVTVSSASTKGPSVFPLAPSSKSTSGGTAALGCLVKDYFPEPVTVSWNSGALTSGVHTFPAVLQSSGLYSLSSVVTVPSSSLGTQTYICNVNHKPSNTKVDKKVEPKSCDKTHTCPPCPAPELLGPSVFLFPPKPKDTLMISRTPEVTCVVVDVSHEDPEVKFNWYVDGVEVHNAKTKPREEQYNSTYRVVSVLTVLHQDWLNGKEYKCKVSNKALGAPIEKTISKAKGQPREPQVYTLPPSREEMTKNQVSLSCAVKGFYPSDIAVEWESNGQPENNYKTTPPVLDSDGSFFLVSKLTVDKSRWQQGNVFSCSVMHEALHNRFTQKSLSLSPGKGGGGSGGGGSGGGGSGGGGSDIQMTQSPSSLSASVGDRVTITCRASQDIRSNLNWYQQKPGGAVKLLIYYTSRLHSGVPSRFSGSGSGTDYTLTISSLQPEDFATYFCQQSEKLPRTFGGGTKVEIR

SEQ ID NO: 66 - protein, 214 aa, synthetic construct
DIQMTQSPSSLSASVGDRVTITCRASQDVNTAVAWYQQKPGKDPKLLIYSASFLYSGVPSRFSGSRSGTDFTLTISSLQPEDFATYYCQQHYTTPPTFGRGTKVEIKRTVAAPSVFIFPPSDEQLKSGTADVVCLLNNFYPREAKVQWKVDNALQSGNSQECVTEQDSKDSTYDLSSTLTLSKADYEKHKVYACEVTHQGLSSPVTKSFNRGEC

SEQ ID NO: 67 - protein, 742 aa, synthetic construct
QLQLQESGPGLVKPSETLSLTCTVSGGSISSGSYFWGWIRQPPGKGLEWIGSIYYSGITYYNPSLKSRVTISVDTSKNQFSLKLSSVTAADTAVYYCARHDGAVAGLFDYWGQGTLVTVSSASTKGPSVFPLAPSSKSTSGGTAALGCLVKDYFPEPVTVSWNSGALTSGVHTFPAVLQSSGLYSLSSVVTVPSSSLGTQTYICNVNHKPSNTKVDKKVEPKSCGGGGSGGGGSGGGGSGGGGSEVQLVESGGGLVQPGGSLRLSCAASGFTFSTYAMNWVRQAPGKGLEWVGRIRSKYNNYATYYADSVKGRFTISRDDSKNSLYLQMNSLKTEDTAVYYCVRHGNFGNSYVSWFAYWGQGTLVTVSSGGGGSDKTHTCPPCPAPELLGPSVFLFPPKPKDTLMISRTPEVTCVVVDVSHEDPEVKFNWYVDGVEVHNAKTKPREEQYNSTYRVVSVLTVLHQDWLNGKEYKCKVSNKALGAPIEKTISKAKGQPREPQVYTLPPSREEMTKNQVSLWCLVKGFYPSDIAVEWESNGQPENNYKTTPPVLDSDGSFFLYSKLTVDKSRWQQGNVFSCSVMHEALHNHYTQKSLSLSPGKGGGGSGGGGSGGGGSGGGGSQVQLVQSGAEVKKPGASVKVSCKASGYTFTDFWMSWVRQAPGQGLEWMGQIYPNTGTTHSNEKFKGRVTMTRDTSTSTVYMELSSLRSEDTAVYYCARSYHISTTPNWFAYWGQGTLVTVSS

SEQ ID NO: 68 - protein, 710 aa, synthetic construct
QLQLQESGPGLVKPSETLSLTCTVSGGSISSGSYFWGWIRQPPGKGLEWIGSIYYSGITYYNPSLKSRVTISVDTSKNQFSLKLSSVTAADTAVYYCARHDGAVAGLFDYWGQGTLVTVSSASTKGPSVFPLAPSSKSTSGGTAALGCLVKDYFPEPVTVSWNSGALTSGVHTFPAVLQSSGLYSLSSVVTVPSSSLGTQTYICNVNHKPSNTKVDKKVEPKSCGGGGSGGGGSGGGGSGGGGSQAVVTQEPSLTVSPGGTVTLTCRSSTGAVTTSNYANWVQQKPGQAPRGLIGGTNKRAPWTPARFSGSLLGGKAALTITGAQAEDEADYYCALWYSNLWVFGGGTKLTVLGGGGSDKTHTCPPCPAPELLGPSVFLFPPKPKDTLMISRTPEVTCVVVDVSHEDPEVKFNWYVDGVEVHNAKTKPREEQYNSTYRVVSVLTVLHQDWLNGKEYKCKVSNKALGAPIEKTISKAKGQPREPQVYTLPPSREEMTKNQVSLSCAVKGFYPSDIAVEWESNGQPENNYKTTPPVLDSDGSFFLVSKLTVDKSRWQQGNVFSCSVMHEALHNRFTQKSLSLSPGKGGGGSGGGGSGGGGSGGGGSDIQMTQSPSSLSASVGDRVTITCKASQNVYKKLEWYQQKPGKVPKVLIYHTNILQTGVPSRFSGSGSGTDYTLTISSLQPEDVATYYCYQWNSGPTFGGGTKVEIK

SEQ ID NO: 69 - protein, 214 aa, synthetic construct
DIQMTQSPSSLSASVGDRVTITCKASQDVSIGVAWYQQKPGKRPKLLIYSASYRYTGVPSRFSGSGSGTDFTLTISSLQPEDFATYYCQQYYIYPYTFGDGTKVEIKRTVAAPSVFIFPPSDEQLKSGTARVVCLLNNFYPREAKVQWKVDNALQSGNSQESVTEQDSKDSTYRLCSTLTLSKADYEKHKVYACEVTHQGLSSPVTKSFNRGEC

SEQ ID NO: 70 - protein, 984 aa, synthetic construct
QVQLVQSGAEVKKPGASVKVSCKASGYTFTNHIIHWVRQAPGQCLEWMGYINPYPGYHAYNEKFQGRATMTSDTSTSTVYMELSSLRSEDTAVYYCARDGYYRDTDVLDYWGQGTLVTVSSGGGGSGGGGSGGGGSDIQMTQSPSSLSASVGDRVTITCQASQDISNYLNWYQQKPGKAPKLLIYYTSRLHTGVPSRFSGSGSGTDFTFTISSLEPEDIATYYCQQGNTLPWTFGCGTKVEIKSGGGGSEVQLVESGGGLVQPGGSLKLSCAASGFTFNKYAMNWVRQAPGKGLEWVARIRSKYNNYATYYADSVKDRFTISRDDSKNTAYLQMNNLKTEDTAVYYCVRHGNFGNSYISYWAYWGQGTLVTVSSGGGGSGGGGSGGGGSQTVVTQEPSLTVSPGGTVTLTCGSSTGAVTSGNYPNWVQQKPGQAPRGLIGGTKFLAPGTPARFSGSLLGGKAALTLSGVQPEDEAEYYCVLWYSNRWVFGGGTKLTVLGGGGDKTHTCPPCPAPELLGGPSVFLFPPKPKDTLMISRTPEVTCVVVDVSHEDPEVKFNWYVDGVEVHNAKTKPCEEQYGSTYRCVSVLTVLHQDWLNGKEYKCKVSNKALPAPIEKTISKAKGQPREPQVYTLPPSREEMTKNQVSLTCLVKGFYPSDIAVEWESNGQPENNYKTTPPVLDSDGSFFLYSKLTVDKSRWQQGNVFSCSVMHEALHNHYTQKSLSLSPGGGGSGGGGSGGGGSGGGGSGGGGSGGGGSDKTHTCPPCPAPELLGGPSVFLFPPKPKDTLMISRTPEVTCVVVDVSHEDPEVKFNWYVDGVEVHNAKTKPCEEQYGSTYRCVSVLTVLHQDWLNGKEYKCKVSNKALPAPIEKTISKAKGQPREPQVYTLPPSREEMTKNQVSLTCLVKGFYPSDIAVEWESNGQPENNYKTTPPVLDSDGSFFLYSKLTVDKSRWQQGNVFSCSVMHEALHNHYTQKSLSLSPGK

SEQ ID NO: 71 - protein, 452 aa, synthetic construct
EVQLVESGGGLVQPGGSLRLSCAASGFTFNTYAMNWVRQAPGKGLEWVARIRSKYNNYATYYAASVKGRFTISRDDSKNSLYLQMNSLKTEDTAVYYCARHGNFGNSYVSWFAYWGQGTLVTVSSASTKGPSVFPLAPCSRSTSESTAALGCLVKDYFPEPVTVSWNSGALTSGVHTFPAVLQSSGLYSLSSVVTVPSSSLGTKTYTCNVDHKPSNTKVDKRVESKYGPPCPPCPAPEAAGGPSVFLFPPKPKDTLMISRTPEVTCVVVDVSQEDPEVQFNWYVDGVEVHNAKTKPREEQFNSTYRVVSVLTVLHQDWLNGKEYKCKVSNKGLPSSIEKTISKAKGQPREPQVYTLPPSQEEMTKNQVSLTCLVKGFYPSDIAVEWESNGQPENNYKTTPPVLDSDGSFLLYSKLTVDKSRWQEGNVFSCSVMHEALHNHYTQKSLSLSLGK

SEQ ID NO: 72 - protein, 448 aa, synthetic construct
QLQLQESGPGLVKPSETLSLTCTVSGGSISSGSYFWGWIRQPPGKGLEWIGSIYYSGITYYNPSLKSRVTISVDTSKNQFSLKLSSVTAADTAVYYCARHDGAVAGLFDYWGQGTLVTVSSASTKGPSVFPLAPCSRSTSESTAALGCLVKDYFPEPVTVSWNSGALTSGVHTFPAVLQSSGLYSLSSVVTVPSSSLGTKTYTCNVDHKPSNTKVDKRVESKYGPPCPPCPAPEAAGGPSVFLFPPKPKDTLMISRTPEVTCVVVDVSQEDPEVQFNWYVDGVEVHNAKTKPREEQFNSTYRVVSVLTVLHQDWLNGKEYKCKVSNKGLPSSIEKTISKAKGQPREPQVYTLPPSQEEMTKNQVSLTCLVKGFYPSDIAVEWESNGQPENNYKTTPPVLDSDGSFFLYSRLTVDKSRWQEGNVFSCSVMHEALHNHYTQKSLSLSLGK

SEQ ID NO: 73 - protein, 215 aa, synthetic construct
QTVVTQEPSLTVSPGGTVTLTCRSSTGAVTTSNYANWVQQKPGQAPRGLIGGTNKRAPGTPARFSGSLLGGKAALTLSGVQPEDEAEYYCALWYSNLWVFGGGTKLTVLGQPKAAPSVTLFPPSSEELQANKATLVCLISDFYPGAVTVAWKADSSPVKAGVETTTPSKQSNNKYAASSYLSLTPEQWKSHRSYSCQVTHEGSTVEKTVAPTECS

SEQ ID NO: 74 - protein, 735 aa, synthetic construct
EVQLVESGGGLVQPGGSLRLSCAASGFNIKDTYIHWVRQAPGKDLEWVARIYPTNGYTRYADSVKGRFTISADTSKNTAYLQMNSLRAEDTAVYYCSRWGGDGFYAMDYWGRGTLVTVSSASTKGPSVFPLAPSSKSTSGGTAALGCLVRDYFPEPVTVSWNSGALTSGVRTFPACLQSSGLYSLSSVVTVPSSSLGTQTYICNVNHKPSNTKVDKKVEPKSCGGGGSGGGGSGGGGSGGGGSEVQLVESGGGLVQPGGSLRLSCAASGFTFSTYAMNWVRQAPGKGLEWVGRIRSKYNNYATYYADSVKGRFTISRDDSKNSLYLQMNSLKTEDTAVYYCVRHGNFGNSYVSWFAYWGQGTLVTVSSGGGGSDKTHTCPPCPAPELLGPSVFLFPPKPKDTLMISRTPEVTCVVVDVSHEDPEVKFNWYVDGVEVHNAKTKPREEQYNSTYRVVSVLTVLHQDWLNGKEYKCKVSNKALGAPIEKTISKAKGQPREPQVYTLPPSREEMTKNQVSLWCLVKGFYPSDIAVEWESNGQPENNYKTTPPVLDSDGSFFLYSKLTVDKSRWQQGNVFSCSVMHEALHNHYTQKSLSLSPGKGGGGSGGGGSGGGGSGGGGSQVQLVQSGAEVKKPGASVKVSCKASGYTFAGFEMHWVRQAPGQGLEWMGAIDPKTGGTDYNQKFKDRVTMTRDTSISTAYMELSRLRSDDTAVYYCARDLGYFDVWGQGTLVTVSS

SEQ ID NO: 75 - protein, 600 aa, synthetic construct
QVQLVQSGAEVKKPGASVKVSCKASGYTFTNHIIHWVRQAPGQGLEWMGYINPYPGYHAYNEKFQGRATMTSDTSTSTVYMELSSLRSEDTAVYYCARDGYYRDTDVLDYWGQGTLVTVSSASTKGPSVFPLAPSSKSTSGGTAALGCLVKDYFPEPVTVSWNSGALTSGVHTFPAVLQSSGLYSLSSVVTVPSSSLGTQTYICNVNHKPSNTKVDKKVEPKSCGGGGSGGGGSGGGGSGGGGSEVQLVESGGGLVQPGGSLRLSCAASGFTFSTYAMNWVRQAPGKGLEWVGRIRSKYNNYATYYADSVKGRFTISRDDSKNSLYLQMNSLKTEDTAVYYCVRHGNFGNSYVSWFAYWGQGTLVTVSSGGGGSDKTHTCPPCPAPELLGPSVFLFPPKPKDTLMISRTPEVTCVVVDVSHEDPEVKFNWYVDGVEVHNAKTKPREEQYNSTYRVVSVLTVLHQDWLNGKEYKCKVSNKALGAPIEKTISKAKGQPREPQVYTLPPSREEMTKNQVSLWCLVKGFYPSDIAVEWESNGQPENNYKTTPPVLDSDGSFFLYSKLTVDKSRWQQGNVFSCSVMHEALHNHYTQKSLSLSPGK

SEQ ID NO: 76 - protein, 584 aa, synthetic construct
QVQLVQSGAEVKKPGASVKVSCKASGYTFTNHIIHWVRQAPGQGLEWMGYINPYPGYHAYNEKFQGRATMTSDTSTSTVYMELSSLRSEDTAVYYCARDGYYRDTDVLDYWGQGTLVTVSSASTKGPSVFPLAPSSKSTSGGTAALGCLVKDYFPEPVTVSWNSGALTSGVHTFPAVLQSSGLYSLSSVVTVPSSSLGTQTYICNVNHKPSNTKVDKKVEPKSCGGGGSGGGGSGGGGSGGGGSQAVVTQEPSLTVSPGGTVTLTCRSSTGAVTTSNYANWVQQKPGQAPRGLIGGTNKRAPWTPARFSGSLLGGKAALTITGAQAEDEADYYCALWYSNLWVFGGGTKLTVLGGGGSDKTHTCPPCPAPELLGPSVFLFPPKPKDTLMISRTPEVTCVVVDVSHEDPEVKFNWYVDGVEVHNAKTKPREEQYNSTYRVVSVLTVLHQDWLNGKEYKCKVSNKALGAPIEKTISKAKGQPREPQVYTLPPSREEMTKNQVSLSCAVKGFYPSDIAVEWESNGQPENNYKTTPPVLDSDGSFFLVSKLTVDKSRWQQGNVFSCSVMHEALHNRFTQKSLSLSPGK

SEQ ID NO: 77 - protein, 709 aa, synthetic construct
EVQLVESGGGLVQPGGSLRLSCAASGFTFTDYTMDWVRQAPGKRLEWVADVNPNSGGSIYNQRFKGRFTLSVDRSKNTLYLQMNSLRAEDTAVYYCARNLGPSFYFDYWGDGTLVTVSSASTKGPSVFPLAPSSKSTSGGTAALGCLVDDYFPEPVTVSWNSGALTSGVDTCPAVLQSSGLYSLSSVVTVPSSSLGTQTYICNVNHKPSNTKVDKKVEPKSCGGGGSGGGGSGGGGSGGGGSQAVVTQEPSLTVSPGGTVTLTCRSSTGAVTTSNYANWVQQKPGQAPRGLIGGTNKRAPWTPARFSGSLLGGKAALTITGAQAEDEADYYCALWYSNLWVFGGGTKLTVLGGGGSDKTHTCPPCPAPELLGPSVFLFPPKPKDTLMISRTPEVTCVVVDVSHEDPEVKFNWYVDGVEVHNAKTKPREEQYNSTYRVVSVLTVLHQDWLNGKEYKCKVSNKALGAPIEKTISKAKGQPREPQVYTLPPSREEMTKNQVSLSCAVKGFYPSDIAVEWESNGQPENNYKTTPPVLDSDGSFFLVSKLTVDKSRWQQGNVFSCSVMHEALHNRFTQKSLSLSPGKGGGGSGGGGSGGGGSGGGGSDIQMTQSPSSLSASVGDRVTITCRASQDIRSNLNWYQQKPGGAVKLLIYYTSRLHSGVPSRFSGSGSGTDYTLTISSLQPEDFATYFCQQSEKLPRTFGGGTKVEIR

SEQ ID NO: 78 - protein, 586 aa, synthetic construct
QVQLVQSGAEVKKPGASVKVSCKASGYTFTNHIIHWVRQAPGQGLEWMGYINPYPGYHAYNEKFQGRATMTSDTSTSTVYMELSSLRSEDTAVYYCARDGYYRDTDVLDYWGQGTLVTVSSASTKGPSVFPLAPSSKSTSGGTAALGCLVKDYFPEPVTVSWNSGALTSGVHTFPAVLQSSGLYSLSSVVTVPSSSLGTQTYICNVNHKPSNTKVDKKVEPKSCDKTHTCPPCPAPELLGPSVFLFPPKPKDTLMISRTPEVTCVVVDVSHEDPEVKFNWYVDGVEVHNAKTKPREEQYNSTYRVVSVLTVLHQDWLNGKEYKCKVSNKALGAPIEKTISKAKGQPREPQVYTLPPSREEMTKNQVSLWCLVKGFYPSDIAVEWESNGQPENNYKTTPPVLDSDGSFFLYSKLTVDKSRWQQGNVFSCSVMHEALHNHYTQKSLSLSPGKGGGGSGGGGSGGGGSGGGGSQVQLVQSGAEVKKPGASVKVSCKASGYTFAGFEMHWVRQAPGQGLEWMGAIDPKTGGTDYNQKFKDRVTMTRDTSISTAYMELSRLRSDDTAVYYCARDLGYFDVWGQGTLVTVSS

SEQ ID NO: 79 - protein, 577 aa, synthetic construct
QVQLVQSGAEVKKPGASVKVSCKASGYTFTNHIIHWVRQAPGQGLEWMGYINPYPGYHAYNEKFQGRATMTSDTSTSTVYMELSSLRSEDTAVYYCARDGYYRDTDVLDYWGQGTLVTVSSASTKGPSVFPLAPSSKSTSGGTAALGCLVKDYFPEPVTVSWNSGALTSGVHTFPAVLQSSGLYSLSSVVTVPSSSLGTQTYICNVNHKPSNTKVDKKVEPKSCDKTHTCPPCPAPELLGPSVFLFPPKPKDTLMISRTPEVTCVVVDVSHEDPEVKFNWYVDGVEVHNAKTKPREEQYNSTYRVVSVLTVLHQDWLNGKEYKCKVSNKALGAPIEKTISKAKGQPREPQVYTLPPSREEMTKNQVSLSCAVKGFYPSDIAVEWESNGQPENNYKTTPPVLDSDGSFFLVSKLTVDKSRWQQGNVFSCSVMHEALHNRFTQKSLSLSPGKGGGGSGGGGSGGGGSGGGGSDIQMTQSPSSLSASVGDRVTITCRASQDIRSNLNWYQQKPGGAVKLLIYYTSRLHSGVPSRFSGSGSGTDYTLTISSLQPEDFATYFCQQSEKLPRTFGGGTKVEIR

SEQ ID NO: 80 - protein, 214 aa, synthetic construct
DIQMTQSPSSLSASVGDRVTITCRASQDVNTAVAWYQQKPGKDPKLLIYSASFLYSGVPSRFSGSRSGTDFTLTISSLQPEDFATYYCQQHYTTPPTFGRGTKVEIKRTVAAPSVFIFPPSDEQLKSGTADVVCLLNNFYPREAKVQWKVDNALQSGNSCESVTEQDSKDSTYDLSSTLTLSKADYEKHKVYACEVTHQGLSSPVTKSFNRGEC

SEQ ID NO: 81 - protein, 742 aa, synthetic construct
QVQLVQSGAEVKKPGASVKVSCKASGYTFTNHIIHWVRQAPGQGLEWMGYINPYPGYHAYNEKFQGRATMTSDTSTSTVYMELSSLRSEDTAVYYCARDGYYRDTDVLDYWGQGTLVTVSSASTKGPSVFPLAPSSKSTSGGTAALGCLVKDYFPEPVTVSWNSGALTSGVHTFPAVLQSSGLYSLSSVVTVPSSSLGTQTYICNVNHKPSNTKVDKKVEPKSCGGGGSGGGGSGGGGSGGGGSEVQLVESGGGLVQPGGSLRLSCAASGFTFSTYAMNWVRQAPGKGLEWVGRIRSKYNNYATYYADSVKGRFTISRDDSKNSLYLQMNSLKTEDTAVYYCVRHGNFGNSYVSWFAYWGQGTLVTVSSGGGGSDKTHTCPPCPAPELLGPSVFLFPPKPKDTLMISRTPEVTCVVVDVSHEDPEVKFNWYVDGVEVHNAKTKPREEQYNSTYRVVSVLTVLHQDWLNGKEYKCKVSNKALGAPIEKTISKAKGQPREPQVYTLPPSREEMTKNQVSLWCLVKGFYPSDIAVEWESNGQPENNYKTTPPVLDSDGSFFLYSKLTVDKSRWQQGNVFSCSVMHEALHNHYTQKSLSLSPGKGGGGSGGGGSGGGGSGGGGSQVQLVQSGAEVKKPGASVKVSCKASGYTFTDFWMSWVRQAPGQGLEWMGQIYPNTGTTHSNEKFKGRVTMTRDTSTSTVYMELSSLRSEDTAVYYCARSYHISTTPNWFAYWGQGTLVTVSS

SEQ ID NO: 82 - protein, 710 aa, synthetic construct
QVQLVQSGAEVKKPGASVKVSCKASGYTFTNHIIHWVRQAPGQGLEWMGYINPYPGYHAYNEKFQGRATMTSDTSTSTVYMELSSLRSEDTAVYYCARDGYYRDTDVLDYWGQGTLVTVSSASTKGPSVFPLAPSSKSTSGGTAALGCLVKDYFPEPVTVSWNSGALTSGVHTFPAVLQSSGLYSLSSVVTVPSSSLGTQTYICNVNHKPSNTKVDKKVEPKSCGGGGSGGGGSGGGGSGGGGSQAVVTQEPSLTVSPGGTVTLTCRSSTGAVTTSNYANWVQQKPGQAPRGLIGGTNKRAPWTPARFSGSLLGGKAALTITGAQAEDEADYYCALWYSNLWVFGGGTKLTVLGGGGSDKTHTCPPCPAPELLGPSVFLFPPKPKDTLMISRTPEVTCVVVDVSHEDPEVKFNWYVDGVEVHNAKTKPREEQYNSTYRVVSVLTVLHQDWLNGKEYKCKVSNKALGAPIEKTISKAKGQPREPQVYTLPPSREEMTKNQVSLSCAVKGFYPSDIAVEWESNGQPENNYKTTPPVLDSDGSFFLVSKLTVDKSRWQQGNVFSCSVMHEALHNRFTQKSLSLSPGKGGGGSGGGGSGGGGSGGGGSDIQMTQSPSSLSASVGDRVTITCKASQNVYKKLEWYQQKPGKVPKVLIYHTNILQTGVPSRFSGSGSGTDYTLTISSLQPEDVATYYCYQWNSGPTFGGGTKVEIK

SEQ ID NO: 83 - protein, 214 aa, synthetic construct
DIQMTQSPSSLSASVGDRVTITCKASQDVSIGVAWYQQKPGKRPKLLIYSASYRYTGVPSRFSGSGSGTDFTLTISSLQPEDFATYYCQQYYIYPYTFGDGTKVEIKRTVAAPSVFIFPPSDEQLKSGTARVVCLLNNFYPREAKVQWKVDNALQSGNSQECVTEQDSKDSTYRLSSTLTLSKADYEKHKVYACEVTHQGLSSPVTKSFNRGEC

SEQ ID NO: 84 - protein, 736 aa, synthetic construct
QVQLVQSGAEVKKPGASVKVSCKASGYTFTSYVMHWVRQKPGQGLEWIGYINPYNEGTESTDKFKGRATMTSDKSTSTVYMELSSLRSEDTAVYYCASIYYGYEGTYFGVWGQGTLVTVSSASTKGPSVFPLAPSSKSTSGGTAALGCLVKDYFPEPVTVSWNSGALTSGVHTFPAVLQSSGLYSLSSVVTVPSSSLGTQTYICNVNHKPSNTKVDKKVEPKSCGGGGSGGGGSGGGGSGGGGSEVQLVESGGGLVQPGGSLRLSCAASGFTFSTYAMNWVRQAPGKGLEWVGRIRSKYNNYATYYADSVKGRFTISRDDSKNSLYLQMNSLKTEDTAVYYCVRHGNFGNSYVSWFAYWGQGTLVTVSSGGGGSDKTHTCPPCPAPELLGPSVFLFPPKPKDTLMISRTPEVTCVVVDVSHEDPEVKFNWYVDGVEVHNAKTKPREEQYNSTYRVVSVLTVLHQDWLNGKEYKCKVSNKALGAPIEKTISKAKGQPREPQVYTLPPSREEMTKNQVSLWCLVKGFYPSDIAVEWESNGQPENNYKTTPPVLDSDGSFFLYSKLTVDKSRWQQGNVFSCSVMHEALHNHYTQKSLSLSPGKGGGGSGGGGSGGGGSGGGGSQVQLVQSGAEVKKPGASVKVSCKASGYTFAGFEMHWVRQAPGQGLEWMGAIDPKTGGTDYNQKFKDRVTMTRDTSISTAYMELSRLRSDDTAVYYCARDLGYFDVWGQGTLVTVSS

SEQ ID NO: 85 - protein, 711 aa, synthetic construct
QVQLVQSGAEVKKPGASVKVSCKASGYTFTSYVMHWVRQKPGQGLEWIGYINPYNEGTESTDKFKGRATMTSDKSTSTVYMELSSLRSEDTAVYYCASIYYGYEGTYFGVWGQGTLVTVSSASTKGPSVFPLAPSSKSTSGGTAALGCLVKDYFPEPVTVSWNSGALTSGVHTFPAVLQSSGLYSLSSVVTVPSSSLGTQTYICNVNHKPSNTKVDKKVEPKSCGGGGSGGGGSGGGGSGGGGSQAVVTQEPSLTVSPGGTVTLTCRSSTGAVTTSNYANWVQQKPGQAPRGLIGGTNKRAPWTPARFSGSLLGGKAALTITGAQAEDEADYYCALWYSNLWVFGGGTKLTVLGGGGSDKTHTCPPCPAPELLGPSVFLFPPKPKDTLMISRTPEVTCVVVDVSHEDPEVKFNWYVDGVEVHNAKTKPREEQYNSTYRVVSVLTVLHQDWLNGKEYKCKVSNKALGAPIEKTISKAKGQPREPQVYTLPPSREEMTKNQVSLSCAVKGFYPSDIAVEWESNGQPENNYKTTPPVLDSDGSFFLVSKLTVDKSRWQQGNVFSCSVMHEALHNHYTQKSLSLSPGKGGGGSGGGGSGGGGSGGGGSDIQMTQSPSSLSASVGDRVTITCRASQDIRSNLNWYQQKPGGAVKLLIYYTSRLHSGVPSRFSGSGSGTDYTLTISSLQPEDFATYFCQQSEKLPRTFGGGTKVEIR

SEQ ID NO: 86 - protein, 213 aa, synthetic construct
EIVLTQSPATLSLSPGERATLSCRASSSVSYMHWYQQKPGQAPRPWIYATSNLASGIPARFSGSRSGTDYTLTISSLEPEDFAVYYCQQWSSNTLTFGGGTKVEIKRTVAAPSVFIFPPSDEQLKSGTASVVCLLNNFYPREAKVQWKVDNALQSGNSQESVTEQDSKDSTYSLSSTLTLSKADYEKHKVYACEVTHQGLSSPVTKSFNRGEC

SEQ ID NO: 87 - protein, 739 aa, synthetic construct
QVQLQQSGAELVRPGSSVKISCKASGYAFSSYWMNWVKQRPGQGLEWIGQIWPGDGDTNYNGKFKGKATLTADESSSTAYMQLSSLASEDSAVYFCARRETTTVGRYYYAMDYWGQGTTVTVSSASTKGPSVFPLAPSSKSTSGGTAALGCLVKDYFPEPVTVSWNSGALTSGVHTFPAVLQSSGLYSLSSVVTVPSSSLGTQTYICNVNHKPSNTKVDKKVEPKSCGGGGSGGGGSGGGGSGGGGSEVQLVESGGGLVQPGGSLRLSCAASGFTFSTYAMNWVRQAPGKGLEWVGRIRSKYNNYATYYADSVKGRFTISRDDSKNSLYLQMNSLKTEDTAVYYCVRHGNFGNSYVSWFAYWGQGTLVTVSSGGGGSDKTHTCPPCPAPELLGPSVFLFPPKPKDTLMISRTPEVTCVVVDVSHEDPEVKFNWYVDGVEVHNAKTKPREEQYNSTYRVVSVLTVLHQDWLNGKEYKCKVSNKALGAPIEKTISKAKGQPREPQVYTLPPSREEMTKNQVSLWCLVKGFYPSDIAVEWESNGQPENNYKTTPPVLDSDGSFFLYSKLTVDKSRWQQGNVFSCSVMHEALHNHYTQKSLSLSPGKGGGGSGGGGSGGGGSGGGGSQVQLVQSGAEVKKPGASVKVSCKASGYTFAGFEMHWVRQAPGQGLEWMGAIDPKTGGTDYNQKFKDRVTMTRDTSISTAYMELSRLRSDDTAVYYCARDLGYFDVWGQGTLVTVSS

SEQ ID NO: 88 - protein, 714 aa, synthetic construct
QVQLQQSGAELVRPGSSVKISCKASGYAFSSYWMNWVKQRPGQGLEWIGQIWPGDGDTNYNGKFKGKATLTADESSSTAYMQLSSLASEDSAVYFCARRETTTVGRYYYAMDYWGQGTTVTVSSASTKGPSVFPLAPSSKSTSGGTAALGCLVKDYFPEPVTVSWNSGALTSGVHTFPAVLQSSGLYSLSSVVTVPSSSLGTQTYICNVNHKPSNTKVDKKVEPKSCGGGGSGGGGSGGGGSGGGGSQAVVTQEPSLTVSPGGTVTLTCRSSTGAVTTSNYANWVQQKPGQAPRGLIGGTNKRAPWTPARFSGSLLGGKAALTITGAQAEDEADYYCALWYSNLWVFGGGTKLTVLGGGGSDKTHTCPPCPAPELLGPSVFLFPPKPKDTLMISRTPEVTCVVVDVSHEDPEVKFNWYVDGVEVHNAKTKPREEQYNSTYRVVSVLTVLHQDWLNGKEYKCKVSNKALGAPIEKTISKAKGQPREPQVYTLPPSREEMTKNQVSLSCAVKGFYPSDIAVEWESNGQPENNYKTTPPVLDSDGSFFLVSKLTVDKSRWQQGNVFSCSVMHEALHNHYTQKSLSLSPGKGGGGSGGGGSGGGGSGGGGSDIQMTQSPSSLSASVGDRVTITCRASQDIRSNLNWYQQKPGGAVKLLIYYTSRLHSGVPSRFSGSGSGTDYTLTISSLQPEDFATYFCQQSEKLPRTFGGGTKVEIR

SEQ ID NO: 89 - protein, 218 aa, synthetic construct
DIQLTQSPASLAVSLGQRATISCKASQSVDYDGDSYLNWYQQIPGQPPKLLIYDASNLVSGIPPRFSGSGSGTDFTLNIHPVEKVDAATYHCQQSTEDPWTFGGGTKLEIKRTVAAPSVFIFPPSDEQLKSGTASVVCLLNNFYPREAKVQWKVDNALQSGNSQESVTEQDSKDSTYSLSSTLTLSKADYEKHKVYACEVTHQGLSSPVTKSFNRGEC

SEQ ID NO: 90 - protein, 102 aa, synthetic construct
SVFLFPPKPKDTLMISRTPEVTCVVVDVSHEDPEVKFNWYVDGVEVHNAKTKPREEQYNSTYRVVSVLTVLHQDWLNGKEYKCKVSNKALPAPIEKTISKAK

SEQ ID NO: 91 - protein, 119 aa, synthetic construct
DKTHTCPPCPAPELLGPSVFLFPPKPKDTLMISRTPEVTCVVVDVSHEDPEVKFNWYVDGVEVHNAKTKPREEQYNSTYRVVSVLTVLHQDWLNGKEYKCKVSNKALGAPIEKTISKAK

SEQ ID NO: 92 - protein, 106 aa, synthetic construct
GQPREPQVYTLPPSREEMTKNQVSLTCLVKGFYPSDIAVEWESNGQPENNYKTTPPVLDSDGSFFLYSKLTVDKSRWQQGNVFSCSVMHEALHNHYTQKSLSLSPG

SEQ ID NO: 93 - protein, 106 aa, synthetic construct
GQPREPQVYTLPPSREEMTKNQVSLWCLVKGFYPSDIAVEWESNGQPENNYKTTPPVLDSDGSFFLYSKLTVDKSRWQQGNVFSCSVMHEALHNHYTQKSLSLSPG

SEQ ID NO: 94 - protein, 106 aa, synthetic construct
GQPREPQVYTLPPSREEMTKNQVSLSCAVKGFYPSDIAVEWESNGQPENNYKTTPPVLDSDGSFFLVSKLTVDKSRWQQGNVFSCSVMHEALHNRFTQKSLSLSPG

SEQ ID NO: 95 - protein, 106 aa, synthetic construct
GQPREPQVYTLPPSREEMTKNQVSLSCAVKGFYPSDIAVEWESNGQPENNYKTTPPVLDSDGSFFLVSKLTVDKSRWQQGNVFSCSVMHEALHNHYTQKSLSLSPG

SEQ ID NO: 96 - protein, 5 aa, synthetic construct
GGGGS

SEQ ID NO: 97 - protein, 10 aa, synthetic construct
GGGGSGGGGS

SEQ ID NO: 98 - protein, 15 aa, synthetic construct
GGGGSGGGGSGGGGS

SEQ ID NO: 99 - protein, 20 aa, synthetic construct
GGGGSGGGGSGGGGSGGGGS

SEQ ID NO: 100 - protein, 25 aa, synthetic construct
GGGGSGGGGSGGGGSGGGGSGGGGS

SEQ ID NO: 101 - protein, 22 aa, synthetic construct
GGGGSDKTHTCPPCPAPELLGP

SEQ ID NO: 102 - protein, 709 aa, synthetic construct
EVQLVESGGGLVQPGGSLRLSCAASGFTFTDYTMDWVRQAPGKRLEWVADVNPNSGGSIYNQRFKGRFTLSVDRSKNTLYLQMNSLRAEDTAVYYCARNLGPSFYFDYWGDGTLVTVSSASTKGPSVFPLAPSSKSTSGGTAALGCLVDDYFPEPVTVSWNSGALTSGVDTFPACLQSSGLYSLSSVVTVPSSSLGTQTYICNVNHKPSNTKVDKKVEPKSCGGGGSGGGGSGGGGSGGGGSQAVVTQEPSLTVSPGGTVTLTCRSSTGAVTTSNYANWVQQKPGQAPRGLIGGTNKRAPWTPARFSGSLLGGKAALTITGAQAEDEADYYCALWYSNLWVFGGGTKLTVLGGGGSDKTHTCPPCPAPELLGPSVFLFPPKPKDTLMISRTPEVTCVVVDVSHEDPEVKFNWYVDGVEVHNAKTKPREEQYNSTYRVVSVLTVLHQDWLNGKEYKCKVSNKALGAPIEKTISKAKGQPREPQVYTLPPSREEMTKNQVSLSCAVKGFYPSDIAVEWESNGQPENNYKTTPPVLDSDGSFFLVSKLTVDKSRWQQGNVFSCSVMHEALHNRFTQKSLSLSPGKGGGGSGGGGSGGGGSGGGGSDIQMTQSPSSLSASVGDRVTITCRASQDIRSNLNWYQQKPGGAVKLLIYYTSRLHSGVPSRFSGSGSGTDYTLTISSLQPEDFATYFCQQSEKLPRTFGGGTKVEIR

SEQ ID NO: 103 - protein, 214 aa, synthetic construct
DIQMTQSPSSLSASVGDRVTITCRASQDVNTAVAWYQQKPGKDPKLLIYSASFLYSGVPSRFSGSRSGTDFTLTISSLQPEDFATYYCQQHYTTPPTFGRGTKVEIKRTVAAPSVFIFPPSDEQLKSGTADVVCLLNNFYPREAKVQWKVDNALQSGNSQESVTEQDSKDSTYDLCSTLTLSKADYEKHKVYACEVTHQGLSSPVTKSFNRGEC

SEQ ID NO: 104 - protein, 214 aa, synthetic construct
DIQMTQSPSSLSASVGDRVTITCKASQDVSIGVAWYQQKPGKRPKLLIYSASYRYTGVPSRFSGSGSGTDFTLTISSLQPEDFATYYCQQYYIYPYTFGDGTKVEIKRTVAAPSVFIFPPSDEQLKSGTARVVCLLNNFYPREAKVQWKVDNALQSGNSCESVTEQDSKDSTYRLSSTLTLSKADYEKHKVYACEVTHQGLSSPVTKSFNRGEC

SEQ ID NO: 105 - protein, 741 aa, synthetic construct
EVQLVESGGGLVQPGGSLRLSCAASGFNIKDTYIHWVRQAPGKDLEWVARIYPTNGYTRYADSVKGRFTISADTSKNTAYLQMNSLRAEDTAVYYCSRWGGDGFYAMDYWGRGTLVTVSSASTKGPSVFPLAPSSKSTSGGTAALGCLVRDYFPEPVTVSWNSGALTSGVRTCPAVLQSSGLYSLSSVVTVPSSSLGTQTYICNVNHKPSNTKVDKKVEPKSCGGGGSGGGGSGGGGSGGGGSEVQLVESGGGLVQPGGSLRLSCAASGFTFSTYAMNWVRQAPGKGLEWVGRIRSKYNNYATYYADSVKGRFTISRDDSKNSLYLQMNSLKTEDTAVYYCVRHGNFGNSYVSWFAYWGQGTLVTVSSGGGGSDKTHTCPPCPAPELLGPSVFLFPPKPKDTLMISRTPEVTCVVVDVSHEDPEVKFNWYVDGVEVHNAKTKPREEQYNSTYRVVSVLTVLHQDWLNGKEYKCKVSNKALGAPIEKTISKAKGQPREPQVYTLPPSREEMTKNQVSLWCLVKGFYPSDIAVEWESNGQPENNYKTTPPVLDSDGSFFLYSKLTVDKSRWQQGNVFSCSVMHEALHNHYTQKSLSLSPGKGGGGSGGGGSGGGGSGGGGSQVQLVQSGAEVKKPGASVKVSCKASGYTFTDFWMSWVRQAPGQGLEWMGQIYPNTGTTHSNEKFKGRVTMTRDTSTSTVYMELSSLRSEDTAVYYCARSYHISTTPNWFAYWGQGTLVTVSS

SEQ ID NO: 106 - protein, 708 aa, synthetic construct
EVQLVESGGGLVQPGGSLRLSCAASGFTFTDYTMDWVRQAPGKRLEWVADVNPNSGGSIYNQRFKGRFTLSVDRSKNTLYLQMNSLRAEDTAVYYCARNLGPSFYFDYWGDGTLVTVSSASTKGPSVFPLAPSSKSTSGGTAALGCLVDDYFPEPVTVSWNSGALTSGVDTFPAVLQSSGLYSLCSVVTVPSSSLGTQTYICNVNHKPSNTKVDKKVEPKSCGGGGSGGGGSGGGGSGGGGSQAVVTQEPSLTVSPGGTVTLTCRSSTGAVTTSNYANWVQQKPGQAPRGLIGGTNKRAPWTPARFSGSLLGGKAALTITGAQAEDEADYYCALWYSNLWVFGGGTKLTVLGGGGSDKTHTCPPCPAPELLGPSVFLFPPKPKDTLMISRTPEVTCVVVDVSHEDPEVKFNWYVDGVEVHNAKTKPREEQYNSTYRVVSVLTVLHQDWLNGKEYKCKVSNKALGAPIEKTISKAKGQPREPQVYTLPPSREEMTKNQVSLSCAVKGFYPSDIAVEWESNGQPENNYKTTPPVLDSDGSFFLVSKLTVDKSRWQQGNVFSCSVMHEALHNRFTQKSLSLSPGKGGGGSGGGGSGGGGSGGGGSDIQMTQSPSSLSASVGDRVTITCKASQNVYKKLEWYQQKPGKVPKVLIYHTNILQTGVPSRFSGSGSGTDYTLTISSLQPEDVATYYCYQWNSGPTFGGGTKVEIK

SEQ ID NO: 107 - protein, 741 aa, synthetic construct
EVQLVESGGGLVQPGGSLRLSCAASGFNIKDTYIHWVRQAPGKDLEWVARIYPTNGYTRYADSVKGRFTISADTSKNTAYLQMNSLRAEDTAVYYCSRWGGDGFYAMDYWGRGTLVTVSSASTKGPSVFPLAPSSKSTSGGTAALGCLVRDYFPEPVTVSWNSGALTSGVRTFPACLQSSGLYSLSSVVTVPSSSLGTQTYICNVNHKPSNTKVDKKVEPKSCGGGGSGGGGSGGGGSGGGGSEVQLVESGGGLVQPGGSLRLSCAASGFTFSTYAMNWVRQAPGKGLEWVGRIRSKYNNYATYYADSVKGRFTISRDDSKNSLYLQMNSLKTEDTAVYYCVRHGNFGNSYVSWFAYWGQGTLVTVSSGGGGSDKTHTCPPCPAPELLGPSVFLFPPKPKDTLMISRTPEVTCVVVDVSHEDPEVKFNWYVDGVEVHNAKTKPREEQYNSTYRVVSVLTVLHQDWLNGKEYKCKVSNKALGAPIEKTISKAKGQPREPQVYTLPPSREEMTKNQVSLWCLVKGFYPSDIAVEWESNGQPENNYKTTPPVLDSDGSFFLYSKLTVDKSRWQQGNVFSCSVMHEALHNHYTQKSLSLSPGKGGGGSGGGGSGGGGSGGGGSQVQLVQSGAEVKKPGASVKVSCKASGYTFTDFWMSWVRQAPGQGLEWMGQIYPNTGTTHSNEKFKGRVTMTRDTSTSTVYMELSSLRSEDTAVYYCARSYHISTTPNWFAYWGQGTLVTVSS

SEQ ID NO: 108 - protein, 708 aa, synthetic construct
EVQLVESGGGLVQPGGSLRLSCAASGFTFTDYTMDWVRQAPGKRLEWVADVNPNSGGSIYNQRFKGRFTLSVDRSKNTLYLQMNSLRAEDTAVYYCARNLGPSFYFDYWGDGTLVTVSSASTKGPSVFPLAPSSKSTSGGTAALGCLVDDYFPEPVTVSWNSGALTSGVDTCPAVLQSSGLYSLSSVVTVPSSSLGTQTYICNVNHKPSNTKVDKKVEPKSCGGGGSGGGGSGGGGSGGGGSQAVVTQEPSLTVSPGGTVTLTCRSSTGAVTTSNYANWVQQKPGQAPRGLIGGTNKRAPWTPARFSGSLLGGKAALTITGAQAEDEADYYCALWYSNLWVFGGGTKLTVLGGGGSDKTHTCPPCPAPELLGPSVFLFPPKPKDTLMISRTPEVTCVVVDVSHEDPEVKFNWYVDGVEVHNAKTKPREEQYNSTYRVVSVLTVLHQDWLNGKEYKCKVSNKALGAPIEKTISKAKGQPREPQVYTLPPSREEMTKNQVSLSCAVKGFYPSDIAVEWESNGQPENNYKTTPPVLDSDGSFFLVSKLTVDKSRWQQGNVFSCSVMHEALHNRFTQKSLSLSPGKGGGGSGGGGSGGGGSGGGGSDIQMTQSPSSLSASVGDRVTITCKASQNVYKKLEWYQQKPGKVPKVLIYHTNILQTGVPSRFSGSGSGTDYTLTISSLQPEDVATYYCYQWNSGPTFGGGTKVEIK

SEQ ID NO: 109 - protein, 708 aa, synthetic construct
EVQLVESGGGLVQPGGSLRLSCAASGFTFTDYTMDWVRQAPGKRLEWVADVNPNSGGSIYNQRFKGRFTLSVDRSKNTLYLQMNSLRAEDTAVYYCARNLGPSFYFDYWGDGTLVTVSSASTKGPSVFPLAPSSKSTSGGTAALGCLVDDYFPEPVTVSWNSGALTSGVDTFPACLQSSGLYSLSSVVTVPSSSLGTQTYICNVNHKPSNTKVDKKVEPKSCGGGGSGGGGSGGGGSGGGGSQAVVTQEPSLTVSPGGTVTLTCRSSTGAVTTSNYANWVQQKPGQAPRGLIGGTNKRAPWTPARFSGSLLGGKAALTITGAQAEDEADYYCALWYSNLWVFGGGTKLTVLGGGGSDKTHTCPPCPAPELLGPSVFLFPPKPKDTLMISRTPEVTCVVVDVSHEDPEVKFNWYVDGVEVHNAKTKPREEQYNSTYRVVSVLTVLHQDWLNGKEYKCKVSNKALGAPIEKTISKAKGQPREPQVYTLPPSREEMTKNQVSLSCAVKGFYPSDIAVEWESNGQPENNYKTTPPVLDSDGSFFLVSKLTVDKSRWQQGNVFSCSVMHEALHNRFTQKSLSLSPGKGGGGSGGGGSGGGGSGGGGSDIQMTQSPSSLSASVGDRVTITCKASQNVYKKLEWYQQKPGKVPKVLIYHTNILQTGVPSRFSGSGSGTDYTLTISSLQPEDVATYYCYQWNSGPTFGGGTKVEIK